European Patent Application EP 4 741 503 A1, published May 13, 2026. Title: 一种抑制AGT基因表达的RNAi剂及其应用. Applicant: 石药集团中奇制药技术（石家庄）有限公司. The sequence listing filed with the application follows.

SEQUENCE LISTING (194 sequences)

SEQ ID NO: 1 - RNA, 21 nt, synthetic construct
  source 1..21: mol_type = other RNA
gtcatccacaatgagagtaca

SEQ ID NO: 2 - RNA, 23 nt, synthetic construct
  source 1..23: mol_type = other RNA
tgtactctcattgtggatgacga

SEQ ID NO: 3 - RNA, 21 nt, synthetic construct
  source 1..21: mol_type = other RNA
gtcatccacaatgagagtacc

SEQ ID NO: 4 - RNA, 23 nt, synthetic construct
  source 1..23: mol_type = other RNA
ggtactctcattgtggatgacga

SEQ ID NO: 5 - RNA, 21 nt, synthetic construct
  source 1..21: mol_type = other RNA
cttctaatgagtcgactttga

SEQ ID NO: 6 - RNA, 23 nt, synthetic construct
  source 1..23: mol_type = other RNA
tcaaagtcgactcattagaagaa

SEQ ID NO: 7 - RNA, 23 nt, synthetic construct
  source 1..23: mol_type = other RNA
  modified_base 11..12: mod_base = OTHER; note = 2 prime-O-methyl uridine; note (original language) = 2'-O-甲基尿苷
  modified_base 2: mod_base = OTHER; note = 2 prime fluoroguanosine; note (original language) = 2'-氟代鸟苷
  modified_base 3: mod_base = OTHER; note = 2 prime-O-methyl uridine; note (original language) = 2'-O-甲基尿苷
  modified_base 4: mod_base = OTHER; note = 2 prime-O-methyl adenosine; note (original language) = 2'-O-甲基腺苷
  modified_base 5: mod_base = OTHER; note = 2 prime-O-methyl cytidine; note (original language) = 2'-O-甲基胞苷
  modified_base 6: mod_base = OTHER; note = 2 prime fluorouridine; note (original language) = 2'-氟代尿苷
  modified_base 7: mod_base = OTHER; note = 2 prime-O-methyl cytidine; note (original language) = 2'-O-甲基胞苷
  modified_base 8: mod_base = OTHER; note = 2 prime-O-methyl uridine; note (original language) = 2'-O-甲基尿苷
  modified_base 9: mod_base = OTHER; note = 2 prime-O-methyl cytidine; note (original language) = 2'-O-甲基胞苷
  modified_base 10: mod_base = OTHER; note = 2 prime-O-methyl adenosine; note (original language) = 2'-O-甲基腺苷
  modified_base 1: mod_base = OTHER; note = 2 prime-O-methyl uridine; note (original language) = 2'-O-甲基尿苷
  modified_base 13: mod_base = OTHER; note = 2 prime-O-methyl guanosine; note (original language) = 2'-O-甲基鸟苷
  modified_base 14: mod_base = OTHER; note = 2 prime fluorouridine; note (original language) = 2'-氟代尿苷
  modified_base 15: mod_base = OTHER; note = 2 prime-O-methyl guanosine; note (original language) = 2'-O-甲基鸟苷
  modified_base 16: mod_base = OTHER; note = 2 prime fluoroguanosine; note (original language) = 2'-氟代鸟苷
  modified_base 17: mod_base = OTHER; note = 2 prime-O-methyl adenosine; note (original language) = 2'-O-甲基腺苷
  modified_base 18: mod_base = OTHER; note = 2 prime-O-methyl uridine; note (original language) = 2'-O-甲基尿苷
  modified_base 19: mod_base = OTHER; note = 2 prime-O-methyl guanosine; note (original language) = 2'-O-甲基鸟苷
  modified_base 20: mod_base = OTHER; note = 2 prime-O-methyl adenosine; note (original language) = 2'-O-甲基腺苷
  modified_base 21: mod_base = OTHER; note = 2 prime-O-methyl cytidine; note (original language) = 2'-O-甲基胞苷
  modified_base 22: mod_base = OTHER; note = 2 prime-O-methyl guanosine; note (original language) = 2'-O-甲基鸟苷
  modified_base 23: mod_base = OTHER; note = 2 prime-O-methyl adenosine; note (original language) = 2'-O-甲基腺苷
  misc_feature 2^3: note = phosphorothioate linkage; note (original language) = 硫代磷酸酯连接
  misc_feature 21^22: note = phosphorothioate linkage; note (original language) = 硫代磷酸酯连接
  misc_feature 22^23: note = phosphorothioate linkage; note (original language) = 硫代磷酸酯连接
  misc_feature 1^2: note = phosphorothioate linkage; note (original language) = 硫代磷酸酯连接
tgtactctcattgtggatgacga

SEQ ID NO: 8 - RNA, 21 nt, synthetic construct
  source 1..21: mol_type = other RNA
  modified_base 1: mod_base = OTHER; note = 2 prime-O-methyl guanosine; note (original language) = 2'-O-甲基鸟苷
  modified_base 2: mod_base = OTHER; note = 2 prime-O-methyl uridine; note (original language) = 2'-O-甲基尿苷
  modified_base 3: mod_base = OTHER; note = 2 prime-O-methyl cytidine; note (original language) = 2'-O-甲基胞苷
  modified_base 4: mod_base = OTHER; note = 2 prime-O-methyl adenosine; note (original language) = 2'-O-甲基腺苷
  modified_base 5: mod_base = OTHER; note = 2 prime-O-methyl uridine; note (original language) = 2'-O-甲基尿苷
  modified_base 6: mod_base = OTHER; note = 2 prime-O-methyl cytidine; note (original language) = 2'-O-甲基胞苷
  modified_base 7: mod_base = OTHER; note = 2 prime fluorocytidine; note (original language) = 2'-氟代胞苷
  modified_base 8: mod_base = OTHER; note = 2 prime-O-methyl adenosine; note (original language) = 2'-O-甲基腺苷
  modified_base 9: mod_base = OTHER; note = 2 prime fluorocytidine; note (original language) = 2'-氟代胞苷
  modified_base 10..11: mod_base = OTHER; note = 2 prime fluoroadenosine; note (original language) = 2'-氟代腺苷
  modified_base 12: mod_base = OTHER; note = 2 prime-O-methyl uridine; note (original language) = 2'-O-甲基尿苷
  modified_base 13: mod_base = OTHER; note = 2 prime-O-methyl guanosine; note (original language) = 2'-O-甲基鸟苷
  modified_base 14: mod_base = OTHER; note = 2 prime-O-methyl adenosine; note (original language) = 2'-O-甲基腺苷
  modified_base 15: mod_base = OTHER; note = 2 prime-O-methyl guanosine; note (original language) = 2'-O-甲基鸟苷
  modified_base 16: mod_base = OTHER; note = 2 prime-O-methyl adenosine; note (original language) = 2'-O-甲基腺苷
  modified_base 17: mod_base = OTHER; note = 2 prime-O-methyl guanosine; note (original language) = 2'-O-甲基鸟苷
  modified_base 18: mod_base = OTHER; note = 2 prime-O-methyl uridine; note (original language) = 2'-O-甲基尿苷
  modified_base 19: mod_base = OTHER; note = 2 prime-O-methyl adenosine; note (original language) = 2'-O-甲基腺苷
  modified_base 20: mod_base = OTHER; note = 2 prime-O-methyl cytidine; note (original language) = 2'-O-甲基胞苷
  modified_base 21: mod_base = OTHER; note = 2 prime-O-methyl adenosine; note (original language) = 2'-O-甲基腺苷
  misc_feature 1^2: note = phosphorothioate linkage; note (original language) = 硫代磷酸酯连接
  misc_feature 2^3: note = phosphorothioate linkage; note (original language) = 硫代磷酸酯连接
gtcatccacaatgagagtaca

SEQ ID NO: 9 - RNA, 23 nt, synthetic construct
  source 1..23: mol_type = other RNA
  modified_base 1: mod_base = OTHER; note = 2 prime-O-methyl guanosine; note (original language) = 2'-O-甲基鸟苷
  modified_base 2: mod_base = OTHER; note = 2 prime fluoroguanosine; note (original language) = 2'-氟代鸟苷
  modified_base 3: mod_base = OTHER; note = 2 prime-O-methyl uridine; note (original language) = 2'-O-甲基尿苷
  modified_base 4: mod_base = OTHER; note = 2 prime-O-methyl adenosine; note (original language) = 2'-O-甲基腺苷
  modified_base 5: mod_base = OTHER; note = 2 prime-O-methyl cytidine; note (original language) = 2'-O-甲基胞苷
  modified_base 6: mod_base = OTHER; note = 2 prime-O-methyl uridine; note (original language) = 2'-O-甲基尿苷
  modified_base 7: mod_base = OTHER; note = 2 prime-O-methyl cytidine; note (original language) = 2'-O-甲基胞苷
  modified_base 8: mod_base = OTHER; note = 2 prime-O-methyl uridine; note (original language) = 2'-O-甲基尿苷
  modified_base 9: mod_base = OTHER; note = 2 prime-O-methyl cytidine; note (original language) = 2'-O-甲基胞苷
  modified_base 10: mod_base = OTHER; note = 2 prime-O-methyl adenosine; note (original language) = 2'-O-甲基腺苷
  modified_base 11..12: mod_base = OTHER; note = 2 prime-O-methyl uridine; note (original language) = 2'-O-甲基尿苷
  modified_base 13: mod_base = OTHER; note = 2 prime-O-methyl guanosine; note (original language) = 2'-O-甲基鸟苷
  modified_base 14: mod_base = OTHER; note = 2 prime fluorouridine; note (original language) = 2'-氟代尿苷
  modified_base 15: mod_base = OTHER; note = 2 prime-O-methyl guanosine; note (original language) = 2'-O-甲基鸟苷
  modified_base 16: mod_base = OTHER; note = 2 prime fluoroguanosine; note (original language) = 2'-氟代鸟苷
  modified_base 17: mod_base = OTHER; note = 2 prime-O-methyl adenosine; note (original language) = 2'-O-甲基腺苷
  modified_base 18: mod_base = OTHER; note = 2 prime-O-methyl uridine; note (original language) = 2'-O-甲基尿苷
  modified_base 19: mod_base = OTHER; note = 2 prime-O-methyl guanosine; note (original language) = 2'-O-甲基鸟苷
  modified_base 20: mod_base = OTHER; note = 2 prime-O-methyl adenosine; note (original language) = 2'-O-甲基腺苷
  modified_base 21: mod_base = OTHER; note = 2 prime-O-methyl cytidine; note (original language) = 2'-O-甲基胞苷
  modified_base 22: mod_base = OTHER; note = 2 prime-O-methyl guanosine; note (original language) = 2'-O-甲基鸟苷
  modified_base 23: mod_base = OTHER; note = 2 prime-O-methyl adenosine; note (original language) = 2'-O-甲基腺苷
  misc_difference 1^2: note = phosphorothioate linkage; note (original language) = 硫代磷酸酯连接
  misc_feature 21^22: note = phosphorothioate linkage; note (original language) = 硫代磷酸酯连接
  misc_feature 22^23: note = phosphorothioate linkage; note (original language) = 硫代磷酸酯连接
  misc_feature 2^3: note = phosphorothioate linkage; note (original language) = 硫代磷酸酯连接
ggtactctcattgtggatgacga

SEQ ID NO: 10 - RNA, 21 nt, synthetic construct
  source 1..21: mol_type = other RNA
  modified_base 1: mod_base = OTHER; note = 2 prime-O-methyl guanosine; note (original language) = 2'-O-甲基鸟苷
  modified_base 2: mod_base = OTHER; note = 2 prime-O-methyl uridine; note (original language) = 2'-O-甲基尿苷
  modified_base 3: mod_base = OTHER; note = 2 prime-O-methyl cytidine; note (original language) = 2'-O-甲基胞苷
  modified_base 4: mod_base = OTHER; note = 2 prime-O-methyl adenosine; note (original language) = 2'-O-甲基腺苷
  modified_base 5: mod_base = OTHER; note = 2 prime-O-methyl uridine; note (original language) = 2'-O-甲基尿苷
  modified_base 6: mod_base = OTHER; note = 2 prime-O-methyl cytidine; note (original language) = 2'-O-甲基胞苷
  modified_base 7: mod_base = OTHER; note = 2 prime fluorocytidine; note (original language) = 2'-氟代胞苷
  modified_base 8: mod_base = OTHER; note = 2 prime-O-methyl adenosine; note (original language) = 2'-O-甲基腺苷
  modified_base 9: mod_base = OTHER; note = 2 prime fluorocytidine; note (original language) = 2'-氟代胞苷
  modified_base 10..11: mod_base = OTHER; note = 2 prime fluoroadenosine; note (original language) = 2'-氟代腺苷
  modified_base 12: mod_base = OTHER; note = 2 prime-O-methyl uridine; note (original language) = 2'-O-甲基尿苷
  modified_base 13: mod_base = OTHER; note = 2 prime-O-methyl guanosine; note (original language) = 2'-O-甲基鸟苷
  modified_base 14: mod_base = OTHER; note = 2 prime-O-methyl adenosine; note (original language) = 2'-O-甲基腺苷
  modified_base 15: mod_base = OTHER; note = 2 prime-O-methyl guanosine; note (original language) = 2'-O-甲基鸟苷
  modified_base 16: mod_base = OTHER; note = 2 prime-O-methyl adenosine; note (original language) = 2'-O-甲基腺苷
  modified_base 17: mod_base = OTHER; note = 2 prime-O-methyl guanosine; note (original language) = 2'-O-甲基鸟苷
  modified_base 18: mod_base = OTHER; note = 2 prime-O-methyl uridine; note (original language) = 2'-O-甲基尿苷
  modified_base 19: mod_base = OTHER; note = 2 prime-O-methyl adenosine; note (original language) = 2'-O-甲基腺苷
  modified_base 20..21: mod_base = OTHER; note = 2 prime-O-methyl cytidine; note (original language) = 2'-O-甲基胞苷
  misc_feature 1^2: note = phosphorothioate linkage; note (original language) = 硫代磷酸酯连接
  misc_feature 2^3: note = phosphorothioate linkage; note (original language) = 硫代磷酸酯连接
gtcatccacaatgagagtacc

SEQ ID NO: 11 - RNA, 23 nt, synthetic construct
  source 1..23: mol_type = other RNA
  modified_base 1: mod_base = OTHER; note = 2 prime-O-methyl guanosine; note (original language) = 2'-O-甲基鸟苷
  modified_base 2: mod_base = OTHER; note = 2 prime fluoroadenosine; note (original language) = 2'-氟代腺苷
  modified_base 3: mod_base = OTHER; note = 2 prime-O-methyl adenosine; note (original language) = 2'-O-甲基腺苷
  modified_base 4..5: mod_base = OTHER; note = 2 prime-O-methyl cytidine; note (original language) = 2'-O-甲基胞苷
  modified_base 6: mod_base = OTHER; note = 2 prime-O-methyl uridine; note (original language) = 2'-O-甲基尿苷
  modified_base 7: mod_base = OTHER; note = 2 prime-O-methyl guanosine; note (original language) = 2'-O-甲基鸟苷
  modified_base 8: mod_base = OTHER; note = 2 prime-O-methyl uridine; note (original language) = 2'-O-甲基尿苷
  modified_base 9: mod_base = OTHER; note = 2 prime-O-methyl cytidine; note (original language) = 2'-O-甲基胞苷
  modified_base 10..11: mod_base = OTHER; note = 2 prime-O-methyl adenosine; note (original language) = 2'-O-甲基腺苷
  modified_base 12: mod_base = OTHER; note = 2 prime-O-methyl uridine; note (original language) = 2'-O-甲基尿苷
  modified_base 13: mod_base = OTHER; note = 2 prime-O-methyl cytidine; note (original language) = 2'-O-甲基胞苷
  modified_base 14: mod_base = OTHER; note = 2 prime fluorouridine; note (original language) = 2'-氟代尿苷
  modified_base 15: mod_base = OTHER; note = 2 prime-O-methyl uridine; note (original language) = 2'-O-甲基尿苷
  modified_base 16: mod_base = OTHER; note = 2 prime fluorocytidine; note (original language) = 2'-氟代胞苷
  modified_base 17: mod_base = OTHER; note = 2 prime-O-methyl uridine; note (original language) = 2'-O-甲基尿苷
  modified_base 18: mod_base = OTHER; note = 2 prime-O-methyl cytidine; note (original language) = 2'-O-甲基胞苷
  modified_base 19: mod_base = OTHER; note = 2 prime-O-methyl adenosine; note (original language) = 2'-O-甲基腺苷
  modified_base 20: mod_base = OTHER; note = 2 prime-O-methyl guanosine; note (original language) = 2'-O-甲基鸟苷
  modified_base 21: mod_base = OTHER; note = 2 prime-O-methyl cytidine; note (original language) = 2'-O-甲基胞苷
  modified_base 22: mod_base = OTHER; note = 2 prime-O-methyl adenosine; note (original language) = 2'-O-甲基腺苷
  modified_base 23: mod_base = OTHER; note = 2 prime-O-methyl guanosine; note (original language) = 2'-O-甲基鸟苷
  misc_feature 1^2: note = phosphorothioate linkage; note (original language) = 硫代磷酸酯连接
  misc_feature 2^3: note = phosphorothioate linkage; note (original language) = 硫代磷酸酯连接
  misc_feature 21^22: note = phosphorothioate linkage; note (original language) = 硫代磷酸酯连接
  misc_feature 22^23: note = phosphorothioate linkage; note (original language) = 硫代磷酸酯连接
gaacctgtcaatcttctcagcag

SEQ ID NO: 12 - RNA, 21 nt, synthetic construct
  source 1..21: mol_type = other RNA
  modified_base 1: mod_base = OTHER; note = 2 prime-O-methyl guanosine; note (original language) = 2'-O-甲基鸟苷
  modified_base 2: mod_base = OTHER; note = 2 prime-O-methyl cytidine; note (original language) = 2'-O-甲基胞苷
  modified_base 3: mod_base = OTHER; note = 2 prime-O-methyl uridine; note (original language) = 2'-O-甲基尿苷
  modified_base 4: mod_base = OTHER; note = 2 prime-O-methyl guanosine; note (original language) = 2'-O-甲基鸟苷
  modified_base 5: mod_base = OTHER; note = 2 prime-O-methyl adenosine; note (original language) = 2'-O-甲基腺苷
  modified_base 6: mod_base = OTHER; note = 2 prime-O-methyl guanosine; note (original language) = 2'-O-甲基鸟苷
  modified_base 7: mod_base = OTHER; note = 2 prime fluoroadenosine; note (original language) = 2'-氟代腺苷
  modified_base 8: mod_base = OTHER; note = 2 prime-O-methyl adenosine; note (original language) = 2'-O-甲基腺苷
  modified_base 9: mod_base = OTHER; note = 2 prime fluoroguanosine; note (original language) = 2'-氟代鸟苷
  modified_base 10: mod_base = OTHER; note = 2 prime fluoroadenosine; note (original language) = 2'-氟代腺苷
  modified_base 11: mod_base = OTHER; note = 2 prime fluorouridine; note (original language) = 2'-氟代尿苷
  modified_base 13: mod_base = OTHER; note = 2 prime-O-methyl guanosine; note (original language) = 2'-O-甲基鸟苷
  modified_base 12: mod_base = OTHER; note = 2 prime-O-methyl uridine; note (original language) = 2'-O-甲基尿苷
  modified_base 14: mod_base = OTHER; note = 2 prime-O-methyl adenosine; note (original language) = 2'-O-甲基腺苷
  modified_base 15: mod_base = OTHER; note = 2 prime-O-methyl cytidine; note (original language) = 2'-O-甲基胞苷
  modified_base 16: mod_base = OTHER; note = 2 prime-O-methyl adenosine; note (original language) = 2'-O-甲基腺苷
  modified_base 17..18: mod_base = OTHER; note = 2 prime-O-methyl guanosine; note (original language) = 2'-O-甲基鸟苷
  modified_base 19..20: mod_base = OTHER; note = 2 prime-O-methyl uridine; note (original language) = 2'-O-甲基尿苷
  modified_base 21: mod_base = OTHER; note = 2 prime-O-methyl cytidine; note (original language) = 2'-O-甲基胞苷
  misc_feature 1^2: note = phosphorothioate linkage; note (original language) = 硫代磷酸酯连接
  misc_feature 2^3: note = phosphorothioate linkage; note (original language) = 硫代磷酸酯连接
gctgagaagattgacaggttc

SEQ ID NO: 13 - RNA, 23 nt, synthetic construct
  source 1..23: mol_type = other RNA
  modified_base 1: mod_base = OTHER; note = 2 prime-O-methyl uridine; note (original language) = 2'-O-甲基尿苷
  modified_base 2: mod_base = OTHER; note = 2 prime fluoroguanosine; note (original language) = 2'-氟代鸟苷
  modified_base 3..4: mod_base = OTHER; note = 2 prime-O-methyl adenosine; note (original language) = 2'-O-甲基腺苷
  modified_base 5..6: mod_base = OTHER; note = 2 prime-O-methyl cytidine; note (original language) = 2'-O-甲基胞苷
  modified_base 7: mod_base = OTHER; note = 2 prime-O-methyl uridine; note (original language) = 2'-O-甲基尿苷
  modified_base 8: mod_base = OTHER; note = 2 prime-O-methyl guanosine; note (original language) = 2'-O-甲基鸟苷
  modified_base 9: mod_base = OTHER; note = 2 prime-O-methyl uridine; note (original language) = 2'-O-甲基尿苷
  modified_base 10: mod_base = OTHER; note = 2 prime-O-methyl cytidine; note (original language) = 2'-O-甲基胞苷
  modified_base 11..12: mod_base = OTHER; note = 2 prime-O-methyl adenosine; note (original language) = 2'-O-甲基腺苷
  modified_base 13: mod_base = OTHER; note = 2 prime-O-methyl uridine; note (original language) = 2'-O-甲基尿苷
  modified_base 14: mod_base = OTHER; note = 2 prime fluorocytidine; note (original language) = 2'-氟代胞苷
  modified_base 15: mod_base = OTHER; note = 2 prime-O-methyl uridine; note (original language) = 2'-O-甲基尿苷
  modified_base 16: mod_base = OTHER; note = 2 prime fluorouridine; note (original language) = 2'-氟代尿苷
  modified_base 17: mod_base = OTHER; note = 2 prime-O-methyl cytidine; note (original language) = 2'-O-甲基胞苷
  modified_base 18: mod_base = OTHER; note = 2 prime-O-methyl uridine; note (original language) = 2'-O-甲基尿苷
  modified_base 19: mod_base = OTHER; note = 2 prime-O-methyl cytidine; note (original language) = 2'-O-甲基胞苷
  modified_base 20: mod_base = OTHER; note = 2 prime-O-methyl adenosine; note (original language) = 2'-O-甲基腺苷
  modified_base 21: mod_base = OTHER; note = 2 prime-O-methyl guanosine; note (original language) = 2'-O-甲基鸟苷
  modified_base 22: mod_base = OTHER; note = 2 prime-O-methyl cytidine; note (original language) = 2'-O-甲基胞苷
  modified_base 23: mod_base = OTHER; note = 2 prime-O-methyl adenosine; note (original language) = 2'-O-甲基腺苷
  misc_feature 1^2: note = phosphorothioate linkage; note (original language) = 硫代磷酸酯连接
  misc_feature 2^3: note = phosphorothioate linkage; note (original language) = 硫代磷酸酯连接
  misc_feature 21^22: note = phosphorothioate linkage; note (original language) = 硫代磷酸酯连接
  misc_feature 22^23: note = phosphorothioate linkage; note (original language) = 硫代磷酸酯连接
tgaacctgtcaatcttctcagca

SEQ ID NO: 14 - RNA, 21 nt, synthetic construct
  source 1..21: mol_type = other RNA
  modified_base 1: mod_base = OTHER; note = 2 prime-O-methyl cytidine; note (original language) = 2'-O-甲基胞苷
  modified_base 2: mod_base = OTHER; note = 2 prime-O-methyl uridine; note (original language) = 2'-O-甲基尿苷
  modified_base 3: mod_base = OTHER; note = 2 prime-O-methyl guanosine; note (original language) = 2'-O-甲基鸟苷
  modified_base 4: mod_base = OTHER; note = 2 prime-O-methyl adenosine; note (original language) = 2'-O-甲基腺苷
  modified_base 5: mod_base = OTHER; note = 2 prime-O-methyl guanosine; note (original language) = 2'-O-甲基鸟苷
  modified_base 6: mod_base = OTHER; note = 2 prime-O-methyl adenosine; note (original language) = 2'-O-甲基腺苷
  modified_base 7: mod_base = OTHER; note = 2 prime fluoroadenosine; note (original language) = 2'-氟代腺苷
  modified_base 8: mod_base = OTHER; note = 2 prime-O-methyl guanosine; note (original language) = 2'-O-甲基鸟苷
  modified_base 9: mod_base = OTHER; note = 2 prime fluoroadenosine; note (original language) = 2'-氟代腺苷
  modified_base 10..11: mod_base = OTHER; note = 2 prime fluorouridine; note (original language) = 2'-氟代尿苷
  modified_base 12: mod_base = OTHER; note = 2 prime-O-methyl guanosine; note (original language) = 2'-O-甲基鸟苷
  modified_base 13: mod_base = OTHER; note = 2 prime-O-methyl adenosine; note (original language) = 2'-O-甲基腺苷
  modified_base 14: mod_base = OTHER; note = 2 prime-O-methyl cytidine; note (original language) = 2'-O-甲基胞苷
  modified_base 15: mod_base = OTHER; note = 2 prime-O-methyl adenosine; note (original language) = 2'-O-甲基腺苷
  modified_base 16..17: mod_base = OTHER; note = 2 prime-O-methyl guanosine; note (original language) = 2'-O-甲基鸟苷
  modified_base 18..19: mod_base = OTHER; note = 2 prime-O-methyl uridine; note (original language) = 2'-O-甲基尿苷
  modified_base 20: mod_base = OTHER; note = 2 prime-O-methyl cytidine; note (original language) = 2'-O-甲基胞苷
  modified_base 21: mod_base = OTHER; note = 2 prime-O-methyl adenosine; note (original language) = 2'-O-甲基腺苷
  misc_feature 1^2: note = phosphorothioate linkage; note (original language) = 硫代磷酸酯连接
  misc_feature 2^3: note = phosphorothioate linkage; note (original language) = 硫代磷酸酯连接
ctgagaagattgacaggttca

SEQ ID NO: 15 - RNA, 23 nt, synthetic construct
  source 1..23: mol_type = other RNA
  modified_base 1: mod_base = OTHER; note = 2 prime-O-methyl uridine; note (original language) = 2'-O-甲基尿苷
  modified_base 2: mod_base = OTHER; note = 2 prime fluoroguanosine; note (original language) = 2'-氟代鸟苷
  modified_base 3: mod_base = OTHER; note = 2 prime-O-methyl adenosine; note (original language) = 2'-O-甲基腺苷
  modified_base 4: mod_base = OTHER; note = 2 prime-O-methyl uridine; note (original language) = 2'-O-甲基尿苷
  modified_base 5: mod_base = OTHER; note = 2 prime-O-methyl cytidine; note (original language) = 2'-O-甲基胞苷
  modified_base 6: mod_base = OTHER; note = 2 prime-O-methyl adenosine; note (original language) = 2'-O-甲基腺苷
  modified_base 7: mod_base = OTHER; note = 2 prime-O-methyl uridine; note (original language) = 2'-O-甲基尿苷
  modified_base 8: mod_base = OTHER; note = 2 prime-O-methyl adenosine; note (original language) = 2'-O-甲基腺苷
  modified_base 9: mod_base = OTHER; note = 2 prime-O-methyl cytidine; note (original language) = 2'-O-甲基胞苷
  modified_base 10: mod_base = OTHER; note = 2 prime-O-methyl adenosine; note (original language) = 2'-O-甲基腺苷
  modified_base 11: mod_base = OTHER; note = 2 prime-O-methyl cytidine; note (original language) = 2'-O-甲基胞苷
  modified_base 12: mod_base = OTHER; note = 2 prime-O-methyl adenosine; note (original language) = 2'-O-甲基腺苷
  modified_base 13: mod_base = OTHER; note = 2 prime-O-methyl guanosine; note (original language) = 2'-O-甲基鸟苷
  modified_base 14: mod_base = OTHER; note = 2 prime fluorocytidine; note (original language) = 2'-氟代胞苷
  modified_base 15: mod_base = OTHER; note = 2 prime-O-methyl adenosine; note (original language) = 2'-O-甲基腺苷
  modified_base 16: mod_base = OTHER; note = 2 prime fluoroadenosine; note (original language) = 2'-氟代腺苷
  modified_base 17: mod_base = OTHER; note = 2 prime-O-methyl adenosine; note (original language) = 2'-O-甲基腺苷
  modified_base 18: mod_base = OTHER; note = 2 prime-O-methyl cytidine; note (original language) = 2'-O-甲基胞苷
  modified_base 19: mod_base = OTHER; note = 2 prime-O-methyl adenosine; note (original language) = 2'-O-甲基腺苷
  modified_base 20..21: mod_base = OTHER; note = 2 prime-O-methyl guanosine; note (original language) = 2'-O-甲基鸟苷
  modified_base 22..23: mod_base = OTHER; note = 2 prime-O-methyl adenosine; note (original language) = 2'-O-甲基腺苷
  misc_feature 1^2: note = phosphorothioate linkage; note (original language) = 硫代磷酸酯连接
  misc_feature 2^3: note = phosphorothioate linkage; note (original language) = 硫代磷酸酯连接
  misc_feature 21^22: note = phosphorothioate linkage; note (original language) = 硫代磷酸酯连接
  misc_feature 22^23: note = phosphorothioate linkage; note (original language) = 硫代磷酸酯连接
tgatcatacacagcaaacaggaa

SEQ ID NO: 16 - RNA, 21 nt, synthetic construct
  source 1..21: mol_type = other RNA
  modified_base 1..2: mod_base = OTHER; note = 2 prime-O-methyl cytidine; note (original language) = 2'-O-甲基胞苷
  modified_base 3: mod_base = OTHER; note = 2 prime-O-methyl uridine; note (original language) = 2'-O-甲基尿苷
  modified_base 4: mod_base = OTHER; note = 2 prime-O-methyl guanosine; note (original language) = 2'-O-甲基鸟苷
  modified_base 5..6: mod_base = OTHER; note = 2 prime-O-methyl uridine; note (original language) = 2'-O-甲基尿苷
  modified_base 7: mod_base = OTHER; note = 2 prime fluorouridine; note (original language) = 2'-氟代尿苷
  modified_base 8: mod_base = OTHER; note = 2 prime-O-methyl guanosine; note (original language) = 2'-O-甲基鸟苷
  modified_base 9: mod_base = OTHER; note = 2 prime fluorocytidine; note (original language) = 2'-氟代胞苷
  modified_base 10: mod_base = OTHER; note = 2 prime fluorouridine; note (original language) = 2'-氟代尿苷
  modified_base 11: mod_base = OTHER; note = 2 prime fluoroguanosine; note (original language) = 2'-氟代鸟苷
  modified_base 12: mod_base = OTHER; note = 2 prime-O-methyl uridine; note (original language) = 2'-O-甲基尿苷
  modified_base 13: mod_base = OTHER; note = 2 prime-O-methyl guanosine; note (original language) = 2'-O-甲基鸟苷
  modified_base 14: mod_base = OTHER; note = 2 prime-O-methyl uridine; note (original language) = 2'-O-甲基尿苷
  modified_base 15: mod_base = OTHER; note = 2 prime-O-methyl adenosine; note (original language) = 2'-O-甲基腺苷
  modified_base 16: mod_base = OTHER; note = 2 prime-O-methyl uridine; note (original language) = 2'-O-甲基尿苷
  modified_base 17: mod_base = OTHER; note = 2 prime-O-methyl guanosine; note (original language) = 2'-O-甲基鸟苷
  modified_base 18: mod_base = OTHER; note = 2 prime-O-methyl adenosine; note (original language) = 2'-O-甲基腺苷
  modified_base 19: mod_base = OTHER; note = 2 prime-O-methyl uridine; note (original language) = 2'-O-甲基尿苷
  modified_base 20: mod_base = OTHER; note = 2 prime-O-methyl cytidine; note (original language) = 2'-O-甲基胞苷
  modified_base 21: mod_base = OTHER; note = 2 prime-O-methyl adenosine; note (original language) = 2'-O-甲基腺苷
  misc_feature 1^2: note = phosphorothioate linkage; note (original language) = 硫代磷酸酯连接
  misc_feature 2^3: note = phosphorothioate linkage; note (original language) = 硫代磷酸酯连接
cctgtttgctgtgtatgatca

SEQ ID NO: 17 - RNA, 23 nt, synthetic construct
  source 1..23: mol_type = other RNA
  modified_base 1: mod_base = OTHER; note = 2 prime-O-methyl uridine; note (original language) = 2'-O-甲基尿苷
  modified_base 2: mod_base = OTHER; note = 2 prime fluoroguanosine; note (original language) = 2'-氟代鸟苷
  modified_base 3: mod_base = OTHER; note = 2 prime-O-methyl adenosine; note (original language) = 2'-O-甲基腺苷
  modified_base 4: mod_base = OTHER; note = 2 prime-O-methyl cytidine; note (original language) = 2'-O-甲基胞苷
  modified_base 5: mod_base = OTHER; note = 2 prime-O-methyl adenosine; note (original language) = 2'-O-甲基腺苷
  modified_base 6: mod_base = OTHER; note = 2 prime-O-methyl cytidine; note (original language) = 2'-O-甲基胞苷
  modified_base 7: mod_base = OTHER; note = 2 prime-O-methyl adenosine; note (original language) = 2'-O-甲基腺苷
  modified_base 8: mod_base = OTHER; note = 2 prime-O-methyl uridine; note (original language) = 2'-O-甲基尿苷
  modified_base 9: mod_base = OTHER; note = 2 prime-O-methyl cytidine; note (original language) = 2'-O-甲基胞苷
  modified_base 10: mod_base = OTHER; note = 2 prime-O-methyl guanosine; note (original language) = 2'-O-甲基鸟苷
  modified_base 11: mod_base = OTHER; note = 2 prime-O-methyl cytidine; note (original language) = 2'-O-甲基胞苷
  modified_base 12: mod_base = OTHER; note = 2 prime-O-methyl uridine; note (original language) = 2'-O-甲基尿苷
  modified_base 13: mod_base = OTHER; note = 2 prime-O-methyl guanosine; note (original language) = 2'-O-甲基鸟苷
  modified_base 14: mod_base = OTHER; note = 2 prime fluoroadenosine; note (original language) = 2'-氟代腺苷
  modified_base 15: mod_base = OTHER; note = 2 prime-O-methyl uridine; note (original language) = 2'-O-甲基尿苷
  modified_base 16: mod_base = OTHER; note = 2 prime fluorouridine; note (original language) = 2'-氟代尿苷
  modified_base 17: mod_base = OTHER; note = 2 prime-O-methyl uridine; note (original language) = 2'-O-甲基尿苷
  modified_base 18: mod_base = OTHER; note = 2 prime-O-methyl guanosine; note (original language) = 2'-O-甲基鸟苷
  modified_base 19: mod_base = OTHER; note = 2 prime-O-methyl uridine; note (original language) = 2'-O-甲基尿苷
  modified_base 20..21: mod_base = OTHER; note = 2 prime-O-methyl cytidine; note (original language) = 2'-O-甲基胞苷
  modified_base 22..23: mod_base = OTHER; note = 2 prime-O-methyl guanosine; note (original language) = 2'-O-甲基鸟苷
  misc_feature 1^2: note = phosphorothioate linkage; note (original language) = 硫代磷酸酯连接
  misc_feature 2^3: note = phosphorothioate linkage; note (original language) = 硫代磷酸酯连接
  misc_feature 21^22: note = phosphorothioate linkage; note (original language) = 硫代磷酸酯连接
  misc_feature 22^23: note = phosphorothioate linkage; note (original language) = 硫代磷酸酯连接
tgacacatcgctgatttgtccgg

SEQ ID NO: 18 - RNA, 21 nt, synthetic construct
  source 1..21: mol_type = other RNA
  modified_base 1..2: mod_base = OTHER; note = 2 prime-O-methyl guanosine; note (original language) = 2'-O-甲基鸟苷
  modified_base 3: mod_base = OTHER; note = 2 prime-O-methyl adenosine; note (original language) = 2'-O-甲基腺苷
  modified_base 4: mod_base = OTHER; note = 2 prime-O-methyl cytidine; note (original language) = 2'-O-甲基胞苷
  modified_base 5..6: mod_base = OTHER; note = 2 prime-O-methyl adenosine; note (original language) = 2'-O-甲基腺苷
  modified_base 7: mod_base = OTHER; note = 2 prime fluoroadenosine; note (original language) = 2'-氟代腺苷
  modified_base 8: mod_base = OTHER; note = 2 prime-O-methyl uridine; note (original language) = 2'-O-甲基尿苷
  modified_base 9: mod_base = OTHER; note = 2 prime fluorocytidine; note (original language) = 2'-氟代胞苷
  modified_base 10: mod_base = OTHER; note = 2 prime fluoroadenosine; note (original language) = 2'-氟代腺苷
  modified_base 11: mod_base = OTHER; note = 2 prime fluoroguanosine; note (original language) = 2'-氟代鸟苷
  modified_base 12: mod_base = OTHER; note = 2 prime-O-methyl cytidine; note (original language) = 2'-O-甲基胞苷
  modified_base 13: mod_base = OTHER; note = 2 prime-O-methyl guanosine; note (original language) = 2'-O-甲基鸟苷
  modified_base 14: mod_base = OTHER; note = 2 prime-O-methyl adenosine; note (original language) = 2'-O-甲基腺苷
  modified_base 15: mod_base = OTHER; note = 2 prime-O-methyl uridine; note (original language) = 2'-O-甲基尿苷
  modified_base 16: mod_base = OTHER; note = 2 prime-O-methyl guanosine; note (original language) = 2'-O-甲基鸟苷
  modified_base 17: mod_base = OTHER; note = 2 prime-O-methyl uridine; note (original language) = 2'-O-甲基尿苷
  modified_base 18: mod_base = OTHER; note = 2 prime-O-methyl guanosine; note (original language) = 2'-O-甲基鸟苷
  modified_base 19: mod_base = OTHER; note = 2 prime-O-methyl uridine; note (original language) = 2'-O-甲基尿苷
  modified_base 21: mod_base = OTHER; note = 2 prime-O-methyl adenosine; note (original language) = 2'-O-甲基腺苷
  modified_base 20: mod_base = OTHER; note = 2 prime-O-methyl cytidine; note (original language) = 2'-O-甲基胞苷
  misc_feature 1^2: note = phosphorothioate linkage; note (original language) = 硫代磷酸酯连接
  misc_feature 2^3: note = phosphorothioate linkage; note (original language) = 硫代磷酸酯连接
ggacaaatcagcgatgtgtca

SEQ ID NO: 19 - RNA, 23 nt, synthetic construct
  source 1..23: mol_type = other RNA
  modified_base 1: mod_base = OTHER; note = 2 prime-O-methyl adenosine; note (original language) = 2'-O-甲基腺苷
  modified_base 2: mod_base = OTHER; note = 2 prime fluoroguanosine; note (original language) = 2'-氟代鸟苷
  modified_base 3..4: mod_base = OTHER; note = 2 prime-O-methyl adenosine; note (original language) = 2'-O-甲基腺苷
  modified_base 5: mod_base = OTHER; note = 2 prime-O-methyl guanosine; note (original language) = 2'-O-甲基鸟苷
  modified_base 6..9: mod_base = OTHER; note = 2 prime-O-methyl adenosine; note (original language) = 2'-O-甲基腺苷
  modified_base 10..11: mod_base = OTHER; note = 2 prime-O-methyl guanosine; note (original language) = 2'-O-甲基鸟苷
  modified_base 12: mod_base = OTHER; note = 2 prime-O-methyl uridine; note (original language) = 2'-O-甲基尿苷
  modified_base 13: mod_base = OTHER; note = 2 prime-O-methyl guanosine; note (original language) = 2'-O-甲基鸟苷
  modified_base 14: mod_base = OTHER; note = 2 prime fluoroguanosine; note (original language) = 2'-氟代鸟苷
  modified_base 15: mod_base = OTHER; note = 2 prime-O-methyl guanosine; note (original language) = 2'-O-甲基鸟苷
  modified_base 16: mod_base = OTHER; note = 2 prime fluoroadenosine; note (original language) = 2'-氟代腺苷
  modified_base 17: mod_base = OTHER; note = 2 prime-O-methyl guanosine; note (original language) = 2'-O-甲基鸟苷
  modified_base 18: mod_base = OTHER; note = 2 prime-O-methyl adenosine; note (original language) = 2'-O-甲基腺苷
  modified_base 19: mod_base = OTHER; note = 2 prime-O-methyl cytidine; note (original language) = 2'-O-甲基胞苷
  modified_base 20: mod_base = OTHER; note = 2 prime-O-methyl uridine; note (original language) = 2'-O-甲基尿苷
  modified_base 21..23: mod_base = OTHER; note = 2 prime-O-methyl guanosine; note (original language) = 2'-O-甲基鸟苷
  misc_feature 1^2: note = phosphorothioate linkage; note (original language) = 硫代磷酸酯连接
  misc_feature 2^3: note = phosphorothioate linkage; note (original language) = 硫代磷酸酯连接
  misc_feature 21^22: note = phosphorothioate linkage; note (original language) = 硫代磷酸酯连接
  misc_feature 22^23: note = phosphorothioate linkage; note (original language) = 硫代磷酸酯连接
agaagaaaaggtgggagactggg

SEQ ID NO: 20 - RNA, 21 nt, synthetic construct
  source 1..21: mol_type = other RNA
  modified_base 1: mod_base = OTHER; note = 2 prime-O-methyl cytidine; note (original language) = 2'-O-甲基胞苷
  modified_base 2: mod_base = OTHER; note = 2 prime-O-methyl adenosine; note (original language) = 2'-O-甲基腺苷
  modified_base 3: mod_base = OTHER; note = 2 prime-O-methyl guanosine; note (original language) = 2'-O-甲基鸟苷
  modified_base 4: mod_base = OTHER; note = 2 prime-O-methyl uridine; note (original language) = 2'-O-甲基尿苷
  modified_base 5: mod_base = OTHER; note = 2 prime-O-methyl cytidine; note (original language) = 2'-O-甲基胞苷
  modified_base 6: mod_base = OTHER; note = 2 prime-O-methyl uridine; note (original language) = 2'-O-甲基尿苷
  modified_base 7: mod_base = OTHER; note = 2 prime fluorocytidine; note (original language) = 2'-氟代胞苷
  modified_base 8: mod_base = OTHER; note = 2 prime-O-methyl cytidine; note (original language) = 2'-O-甲基胞苷
  modified_base 9: mod_base = OTHER; note = 2 prime fluorocytidine; note (original language) = 2'-氟代胞苷
  modified_base 10: mod_base = OTHER; note = 2 prime fluoroadenosine; note (original language) = 2'-氟代腺苷
  modified_base 11: mod_base = OTHER; note = 2 prime fluorocytidine; note (original language) = 2'-氟代胞苷
  modified_base 12: mod_base = OTHER; note = 2 prime-O-methyl cytidine; note (original language) = 2'-O-甲基胞苷
  modified_base 13..16: mod_base = OTHER; note = 2 prime-O-methyl uridine; note (original language) = 2'-O-甲基尿苷
  modified_base 17: mod_base = OTHER; note = 2 prime-O-methyl cytidine; note (original language) = 2'-O-甲基胞苷
  modified_base 18..19: mod_base = OTHER; note = 2 prime-O-methyl uridine; note (original language) = 2'-O-甲基尿苷
  modified_base 20: mod_base = OTHER; note = 2 prime-O-methyl cytidine; note (original language) = 2'-O-甲基胞苷
  modified_base 21: mod_base = OTHER; note = 2 prime-O-methyl uridine; note (original language) = 2'-O-甲基尿苷
  misc_feature 1^2: note = phosphorothioate linkage; note (original language) = 硫代磷酸酯连接
  misc_feature 2^3: note = phosphorothioate linkage; note (original language) = 硫代磷酸酯连接
cagtctcccaccttttcttct

SEQ ID NO: 21 - RNA, 23 nt, synthetic construct
  source 1..23: mol_type = other RNA
  modified_base 1: mod_base = OTHER; note = 2 prime-O-methyl cytidine; note (original language) = 2'-O-甲基胞苷
  modified_base 2: mod_base = OTHER; note = 2 prime fluoroadenosine; note (original language) = 2'-氟代腺苷
  modified_base 3..4: mod_base = OTHER; note = 2 prime-O-methyl uridine; note (original language) = 2'-O-甲基尿苷
  modified_base 5: mod_base = OTHER; note = 2 prime-O-methyl adenosine; note (original language) = 2'-O-甲基腺苷
  modified_base 6: mod_base = OTHER; note = 2 prime-O-methyl guanosine; note (original language) = 2'-O-甲基鸟苷
  modified_base 7..8: mod_base = OTHER; note = 2 prime-O-methyl adenosine; note (original language) = 2'-O-甲基腺苷
  modified_base 9: mod_base = OTHER; note = 2 prime-O-methyl guanosine; note (original language) = 2'-O-甲基鸟苷
  modified_base 10..13: mod_base = OTHER; note = 2 prime-O-methyl adenosine; note (original language) = 2'-O-甲基腺苷
  modified_base 14: mod_base = OTHER; note = 2 prime fluoroguanosine; note (original language) = 2'-氟代鸟苷
  modified_base 15: mod_base = OTHER; note = 2 prime-O-methyl guanosine; note (original language) = 2'-O-甲基鸟苷
  modified_base 16: mod_base = OTHER; note = 2 prime fluorouridine; note (original language) = 2'-氟代尿苷
  modified_base 17..19: mod_base = OTHER; note = 2 prime-O-methyl guanosine; note (original language) = 2'-O-甲基鸟苷
  modified_base 20: mod_base = OTHER; note = 2 prime-O-methyl adenosine; note (original language) = 2'-O-甲基腺苷
  modified_base 21: mod_base = OTHER; note = 2 prime-O-methyl guanosine; note (original language) = 2'-O-甲基鸟苷
  modified_base 22: mod_base = OTHER; note = 2 prime-O-methyl adenosine; note (original language) = 2'-O-甲基腺苷
  modified_base 23: mod_base = OTHER; note = 2 prime-O-methyl cytidine; note (original language) = 2'-O-甲基胞苷
  misc_feature 1^2: note = phosphorothioate linkage; note (original language) = 硫代磷酸酯连接
  misc_feature 2^3: note = phosphorothioate linkage; note (original language) = 硫代磷酸酯连接
  misc_feature 21^22: note = phosphorothioate linkage; note (original language) = 硫代磷酸酯连接
  misc_feature 22^23: note = phosphorothioate linkage; note (original language) = 硫代磷酸酯连接
cattagaagaaaaggtgggagac

SEQ ID NO: 22 - RNA, 21 nt, synthetic construct
  source 1..21: mol_type = other RNA
  modified_base 1: mod_base = OTHER; note = 2 prime-O-methyl cytidine; note (original language) = 2'-O-甲基胞苷
  modified_base 2: mod_base = OTHER; note = 2 prime-O-methyl uridine; note (original language) = 2'-O-甲基尿苷
  modified_base 3..5: mod_base = OTHER; note = 2 prime-O-methyl cytidine; note (original language) = 2'-O-甲基胞苷
  modified_base 6: mod_base = OTHER; note = 2 prime-O-methyl adenosine; note (original language) = 2'-O-甲基腺苷
  modified_base 7: mod_base = OTHER; note = 2 prime fluorocytidine; note (original language) = 2'-氟代胞苷
  modified_base 8: mod_base = OTHER; note = 2 prime-O-methyl cytidine; note (original language) = 2'-O-甲基胞苷
  modified_base 9..11: mod_base = OTHER; note = 2 prime fluorouridine; note (original language) = 2'-氟代尿苷
  modified_base 12: mod_base = OTHER; note = 2 prime-O-methyl uridine; note (original language) = 2'-O-甲基尿苷
  modified_base 13: mod_base = OTHER; note = 2 prime-O-methyl cytidine; note (original language) = 2'-O-甲基胞苷
  modified_base 14..15: mod_base = OTHER; note = 2 prime-O-methyl uridine; note (original language) = 2'-O-甲基尿苷
  modified_base 16: mod_base = OTHER; note = 2 prime-O-methyl cytidine; note (original language) = 2'-O-甲基胞苷
  modified_base 17: mod_base = OTHER; note = 2 prime-O-methyl uridine; note (original language) = 2'-O-甲基尿苷
  modified_base 18..19: mod_base = OTHER; note = 2 prime-O-methyl adenosine; note (original language) = 2'-O-甲基腺苷
  modified_base 20: mod_base = OTHER; note = 2 prime-O-methyl uridine; note (original language) = 2'-O-甲基尿苷
  modified_base 21: mod_base = OTHER; note = 2 prime-O-methyl guanosine; note (original language) = 2'-O-甲基鸟苷
  misc_feature 1^2: note = phosphorothioate linkage; note (original language) = 硫代磷酸酯连接
  misc_feature 2^3: note = phosphorothioate linkage; note (original language) = 硫代磷酸酯连接
ctcccaccttttcttctaatg

SEQ ID NO: 23 - RNA, 23 nt, synthetic construct
  source 1..23: mol_type = other RNA
  modified_base 1: mod_base = OTHER; note = 2 prime-O-methyl uridine; note (original language) = 2'-O-甲基尿苷
  modified_base 2: mod_base = OTHER; note = 2 prime fluorocytidine; note (original language) = 2'-氟代胞苷
  modified_base 3..5: mod_base = OTHER; note = 2 prime-O-methyl adenosine; note (original language) = 2'-O-甲基腺苷
  modified_base 6: mod_base = OTHER; note = 2 prime-O-methyl guanosine; note (original language) = 2'-O-甲基鸟苷
  modified_base 7: mod_base = OTHER; note = 2 prime-O-methyl uridine; note (original language) = 2'-O-甲基尿苷
  modified_base 8: mod_base = OTHER; note = 2 prime-O-methyl cytidine; note (original language) = 2'-O-甲基胞苷
  modified_base 9: mod_base = OTHER; note = 2 prime-O-methyl guanosine; note (original language) = 2'-O-甲基鸟苷
  modified_base 10: mod_base = OTHER; note = 2 prime-O-methyl adenosine; note (original language) = 2'-O-甲基腺苷
  modified_base 11: mod_base = OTHER; note = 2 prime-O-methyl cytidine; note (original language) = 2'-O-甲基胞苷
  modified_base 12: mod_base = OTHER; note = 2 prime-O-methyl uridine; note (original language) = 2'-O-甲基尿苷
  modified_base 13: mod_base = OTHER; note = 2 prime-O-methyl cytidine; note (original language) = 2'-O-甲基胞苷
  modified_base 14: mod_base = OTHER; note = 2 prime fluoroadenosine; note (original language) = 2'-氟代腺苷
  modified_base 15: mod_base = OTHER; note = 2 prime-O-methyl uridine; note (original language) = 2'-O-甲基尿苷
  modified_base 16: mod_base = OTHER; note = 2 prime fluorouridine; note (original language) = 2'-氟代尿苷
  modified_base 17: mod_base = OTHER; note = 2 prime-O-methyl adenosine; note (original language) = 2'-O-甲基腺苷
  modified_base 18: mod_base = OTHER; note = 2 prime-O-methyl guanosine; note (original language) = 2'-O-甲基鸟苷
  modified_base 19..20: mod_base = OTHER; note = 2 prime-O-methyl adenosine; note (original language) = 2'-O-甲基腺苷
  modified_base 21: mod_base = OTHER; note = 2 prime-O-methyl guanosine; note (original language) = 2'-O-甲基鸟苷
  modified_base 22..23: mod_base = OTHER; note = 2 prime-O-methyl adenosine; note (original language) = 2'-O-甲基腺苷
  misc_feature 1^2: note = phosphorothioate linkage; note (original language) = 硫代磷酸酯连接
  misc_feature 2^3: note = phosphorothioate linkage; note (original language) = 硫代磷酸酯连接
  misc_feature 21^22: note = phosphorothioate linkage; note (original language) = 硫代磷酸酯连接
  misc_feature 22^23: note = phosphorothioate linkage; note (original language) = 硫代磷酸酯连接
tcaaagtcgactcattagaagaa

SEQ ID NO: 24 - RNA, 21 nt, synthetic construct
  source 1..21: mol_type = other RNA
  modified_base 1: mod_base = OTHER; note = 2 prime-O-methyl cytidine; note (original language) = 2'-O-甲基胞苷
  modified_base 2..3: mod_base = OTHER; note = 2 prime-O-methyl uridine; note (original language) = 2'-O-甲基尿苷
  modified_base 4: mod_base = OTHER; note = 2 prime-O-methyl cytidine; note (original language) = 2'-O-甲基胞苷
  modified_base 5: mod_base = OTHER; note = 2 prime-O-methyl uridine; note (original language) = 2'-O-甲基尿苷
  modified_base 6: mod_base = OTHER; note = 2 prime-O-methyl adenosine; note (original language) = 2'-O-甲基腺苷
  modified_base 7: mod_base = OTHER; note = 2 prime fluoroadenosine; note (original language) = 2'-氟代腺苷
  modified_base 8: mod_base = OTHER; note = 2 prime-O-methyl uridine; note (original language) = 2'-O-甲基尿苷
  modified_base 9: mod_base = OTHER; note = 2 prime fluoroguanosine; note (original language) = 2'-氟代鸟苷
  modified_base 10: mod_base = OTHER; note = 2 prime fluoroadenosine; note (original language) = 2'-氟代腺苷
  modified_base 11: mod_base = OTHER; note = 2 prime fluoroguanosine; note (original language) = 2'-氟代鸟苷
  modified_base 12: mod_base = OTHER; note = 2 prime-O-methyl uridine; note (original language) = 2'-O-甲基尿苷
  modified_base 13: mod_base = OTHER; note = 2 prime-O-methyl cytidine; note (original language) = 2'-O-甲基胞苷
  modified_base 14: mod_base = OTHER; note = 2 prime-O-methyl guanosine; note (original language) = 2'-O-甲基鸟苷
  modified_base 15: mod_base = OTHER; note = 2 prime-O-methyl adenosine; note (original language) = 2'-O-甲基腺苷
  modified_base 16: mod_base = OTHER; note = 2 prime-O-methyl cytidine; note (original language) = 2'-O-甲基胞苷
  modified_base 17..19: mod_base = OTHER; note = 2 prime-O-methyl uridine; note (original language) = 2'-O-甲基尿苷
  modified_base 20: mod_base = OTHER; note = 2 prime-O-methyl guanosine; note (original language) = 2'-O-甲基鸟苷
  modified_base 21: mod_base = OTHER; note = 2 prime-O-methyl adenosine; note (original language) = 2'-O-甲基腺苷
  misc_feature 1^2: note = phosphorothioate linkage; note (original language) = 硫代磷酸酯连接
  misc_feature 2^3: note = phosphorothioate linkage; note (original language) = 硫代磷酸酯连接
cttctaatgagtcgactttga

SEQ ID NO: 25 - RNA, 23 nt, synthetic construct
  source 1..23: mol_type = other RNA
  modified_base 1: mod_base = OTHER; note = 2 prime-O-methyl adenosine; note (original language) = 2'-O-甲基腺苷
  modified_base 2: mod_base = OTHER; note = 2 prime fluorocytidine; note (original language) = 2'-氟代胞苷
  modified_base 3: mod_base = OTHER; note = 2 prime-O-methyl adenosine; note (original language) = 2'-O-甲基腺苷
  modified_base 4: mod_base = OTHER; note = 2 prime-O-methyl cytidine; note (original language) = 2'-O-甲基胞苷
  modified_base 5..6: mod_base = OTHER; note = 2 prime-O-methyl uridine; note (original language) = 2'-O-甲基尿苷
  modified_base 7: mod_base = OTHER; note = 2 prime-O-methyl adenosine; note (original language) = 2'-O-甲基腺苷
  modified_base 8: mod_base = OTHER; note = 2 prime-O-methyl guanosine; note (original language) = 2'-O-甲基鸟苷
  modified_base 9: mod_base = OTHER; note = 2 prime-O-methyl adenosine; note (original language) = 2'-O-甲基腺苷
  modified_base 10..11: mod_base = OTHER; note = 2 prime-O-methyl cytidine; note (original language) = 2'-O-甲基胞苷
  modified_base 12..13: mod_base = OTHER; note = 2 prime-O-methyl adenosine; note (original language) = 2'-O-甲基腺苷
  modified_base 14: mod_base = OTHER; note = 2 prime fluoroguanosine; note (original language) = 2'-氟代鸟苷
  modified_base 15: mod_base = OTHER; note = 2 prime-O-methyl guanosine; note (original language) = 2'-O-甲基鸟苷
  modified_base 16: mod_base = OTHER; note = 2 prime fluoroadenosine; note (original language) = 2'-氟代腺苷
  modified_base 17: mod_base = OTHER; note = 2 prime-O-methyl guanosine; note (original language) = 2'-O-甲基鸟苷
  modified_base 18..20: mod_base = OTHER; note = 2 prime-O-methyl adenosine; note (original language) = 2'-O-甲基腺苷
  modified_base 21: mod_base = OTHER; note = 2 prime-O-methyl cytidine; note (original language) = 2'-O-甲基胞苷
  modified_base 22..23: mod_base = OTHER; note = 2 prime-O-methyl guanosine; note (original language) = 2'-O-甲基鸟苷
  misc_feature 1^2: note = phosphorothioate linkage; note (original language) = 硫代磷酸酯连接
  misc_feature 2^3: note = phosphorothioate linkage; note (original language) = 硫代磷酸酯连接
  misc_feature 21^22: note = phosphorothioate linkage; note (original language) = 硫代磷酸酯连接
  misc_feature 22^23: note = phosphorothioate linkage; note (original language) = 硫代磷酸酯连接
acacttagaccaaggagaaacgg

SEQ ID NO: 26 - RNA, 21 nt, synthetic construct
  source 1..21: mol_type = other RNA
  modified_base 1: mod_base = OTHER; note = 2 prime-O-methyl guanosine; note (original language) = 2'-O-甲基鸟苷
  modified_base 2..4: mod_base = OTHER; note = 2 prime-O-methyl uridine; note (original language) = 2'-O-甲基尿苷
  modified_base 5: mod_base = OTHER; note = 2 prime-O-methyl cytidine; note (original language) = 2'-O-甲基胞苷
  modified_base 6: mod_base = OTHER; note = 2 prime-O-methyl uridine; note (original language) = 2'-O-甲基尿苷
  modified_base 7: mod_base = OTHER; note = 2 prime fluorocytidine; note (original language) = 2'-氟代胞苷
  modified_base 9: mod_base = OTHER; note = 2 prime-O-methyl cytidine; note (original language) = 2'-O-甲基胞苷
  modified_base 9..10: mod_base = OTHER; note = 2 prime fluorouridine; note (original language) = 2'-氟代尿苷
  modified_base 11: mod_base = OTHER; note = 2 prime fluoroguanosine; note (original language) = 2'-氟代鸟苷
  modified_base 12: mod_base = OTHER; note = 2 prime-O-methyl guanosine; note (original language) = 2'-O-甲基鸟苷
  modified_base 13: mod_base = OTHER; note = 2 prime-O-methyl uridine; note (original language) = 2'-O-甲基尿苷
  modified_base 14: mod_base = OTHER; note = 2 prime-O-methyl cytidine; note (original language) = 2'-O-甲基胞苷
  modified_base 15: mod_base = OTHER; note = 2 prime-O-methyl uridine; note (original language) = 2'-O-甲基尿苷
  modified_base 16..17: mod_base = OTHER; note = 2 prime-O-methyl adenosine; note (original language) = 2'-O-甲基腺苷
  modified_base 18: mod_base = OTHER; note = 2 prime-O-methyl guanosine; note (original language) = 2'-O-甲基鸟苷
  modified_base 19: mod_base = OTHER; note = 2 prime-O-methyl uridine; note (original language) = 2'-O-甲基尿苷
  modified_base 20: mod_base = OTHER; note = 2 prime-O-methyl guanosine; note (original language) = 2'-O-甲基鸟苷
  modified_base 21: mod_base = OTHER; note = 2 prime-O-methyl uridine; note (original language) = 2'-O-甲基尿苷
  misc_feature 1^2: note = phosphorothioate linkage; note (original language) = 硫代磷酸酯连接
  misc_feature 2^3: note = phosphorothioate linkage; note (original language) = 硫代磷酸酯连接
gtttctccttggtctaagtgt

SEQ ID NO: 27 - RNA, 23 nt, synthetic construct
  source 1..23: mol_type = other RNA
  modified_base 1: mod_base = OTHER; note = 2 prime-O-methyl uridine; note (original language) = 2'-O-甲基尿苷
  modified_base 2: mod_base = OTHER; note = 2 prime fluorouridine; note (original language) = 2'-氟代尿苷
  modified_base 3..6: mod_base = OTHER; note = 2 prime-O-methyl uridine; note (original language) = 2'-O-甲基尿苷
  modified_base 7: mod_base = OTHER; note = 2 prime-O-methyl guanosine; note (original language) = 2'-O-甲基鸟苷
  modified_base 8..10: mod_base = OTHER; note = 2 prime-O-methyl uridine; note (original language) = 2'-O-甲基尿苷
  modified_base 11: mod_base = OTHER; note = 2 prime-O-methyl cytidine; note (original language) = 2'-O-甲基胞苷
  modified_base 12: mod_base = OTHER; note = 2 prime-O-methyl adenosine; note (original language) = 2'-O-甲基腺苷
  modified_base 13: mod_base = OTHER; note = 2 prime-O-methyl cytidine; note (original language) = 2'-O-甲基胞苷
  modified_base 14: mod_base = OTHER; note = 2 prime fluoroadenosine; note (original language) = 2'-氟代腺苷
  modified_base 15: mod_base = OTHER; note = 2 prime-O-methyl adenosine; note (original language) = 2'-O-甲基腺苷
  modified_base 16: mod_base = OTHER; note = 2 prime fluoroadenosine; note (original language) = 2'-氟代腺苷
  modified_base 17: mod_base = OTHER; note = 2 prime-O-methyl cytidine; note (original language) = 2'-O-甲基胞苷
  modified_base 18..19: mod_base = OTHER; note = 2 prime-O-methyl adenosine; note (original language) = 2'-O-甲基腺苷
  modified_base 20: mod_base = OTHER; note = 2 prime-O-methyl guanosine; note (original language) = 2'-O-甲基鸟苷
  modified_base 21: mod_base = OTHER; note = 2 prime-O-methyl cytidine; note (original language) = 2'-O-甲基胞苷
  modified_base 22: mod_base = OTHER; note = 2 prime-O-methyl uridine; note (original language) = 2'-O-甲基尿苷
  modified_base 23: mod_base = OTHER; note = 2 prime-O-methyl guanosine; note (original language) = 2'-O-甲基鸟苷
  misc_feature 1^2: note = phosphorothioate linkage; note (original language) = 硫代磷酸酯连接
  misc_feature 2^3: note = phosphorothioate linkage; note (original language) = 硫代磷酸酯连接
  misc_feature 21^22: note = phosphorothioate linkage; note (original language) = 硫代磷酸酯连接
  misc_feature 22^23: note = phosphorothioate linkage; note (original language) = 硫代磷酸酯连接
ttttttgtttcacaaacaagctg

SEQ ID NO: 28 - RNA, 21 nt, synthetic construct
  source 1..21: mol_type = other RNA
  modified_base 1: mod_base = OTHER; note = 2 prime-O-methyl guanosine; note (original language) = 2'-O-甲基鸟苷
  modified_base 2: mod_base = OTHER; note = 2 prime-O-methyl cytidine; note (original language) = 2'-O-甲基胞苷
  modified_base 3..4: mod_base = OTHER; note = 2 prime-O-methyl uridine; note (original language) = 2'-O-甲基尿苷
  modified_base 5: mod_base = OTHER; note = 2 prime-O-methyl guanosine; note (original language) = 2'-O-甲基鸟苷
  modified_base 6: mod_base = OTHER; note = 2 prime-O-methyl uridine; note (original language) = 2'-O-甲基尿苷
  modified_base 7: mod_base = OTHER; note = 2 prime fluorouridine; note (original language) = 2'-氟代尿苷
  modified_base 8: mod_base = OTHER; note = 2 prime-O-methyl uridine; note (original language) = 2'-O-甲基尿苷
  modified_base 9: mod_base = OTHER; note = 2 prime fluoroguanosine; note (original language) = 2'-氟代鸟苷
  modified_base 10: mod_base = OTHER; note = 2 prime fluorouridine; note (original language) = 2'-氟代尿苷
  modified_base 11: mod_base = OTHER; note = 2 prime fluoroguanosine; note (original language) = 2'-氟代鸟苷
  modified_base 12..14: mod_base = OTHER; note = 2 prime-O-methyl adenosine; note (original language) = 2'-O-甲基腺苷
  modified_base 15: mod_base = OTHER; note = 2 prime-O-methyl cytidine; note (original language) = 2'-O-甲基胞苷
  modified_base 16..21: mod_base = OTHER; note = 2 prime-O-methyl adenosine; note (original language) = 2'-O-甲基腺苷
  misc_feature 1^2: note = phosphorothioate linkage; note (original language) = 硫代磷酸酯连接
  misc_feature 2^3: note = phosphorothioate linkage; note (original language) = 硫代磷酸酯连接
gcttgtttgtgaaacaaaaaa

SEQ ID NO: 29 - RNA, 21 nt, synthetic construct
  source 1..21: mol_type = other RNA
  modified_base 1: mod_base = OTHER; note = 2 prime-O-methyl guanosine; note (original language) = 2'-O-甲基鸟苷
  modified_base 2: mod_base = OTHER; note = 2 prime-O-methyl uridine; note (original language) = 2'-O-甲基尿苷
  modified_base 3: mod_base = OTHER; note = 2 prime-O-methyl cytidine; note (original language) = 2'-O-甲基胞苷
  modified_base 4: mod_base = OTHER; note = 2 prime-O-methyl adenosine; note (original language) = 2'-O-甲基腺苷
  modified_base 5: mod_base = OTHER; note = 2 prime-O-methyl uridine; note (original language) = 2'-O-甲基尿苷
  modified_base 6: mod_base = OTHER; note = 2 prime-O-methyl cytidine; note (original language) = 2'-O-甲基胞苷
  modified_base 7: mod_base = OTHER; note = 2 prime fluorocytidine; note (original language) = 2'-氟代胞苷
  modified_base 8: mod_base = OTHER; note = 2 prime-O-methyl adenosine; note (original language) = 2'-O-甲基腺苷
  modified_base 9: mod_base = OTHER; note = 2 prime fluorocytidine; note (original language) = 2'-氟代胞苷
  modified_base 10..11: mod_base = OTHER; note = 2 prime fluoroadenosine; note (original language) = 2'-氟代腺苷
  modified_base 12: mod_base = OTHER; note = 2 prime-O-methyl uridine; note (original language) = 2'-O-甲基尿苷
  modified_base 13: mod_base = OTHER; note = 2 prime-O-methyl guanosine; note (original language) = 2'-O-甲基鸟苷
  modified_base 14: mod_base = OTHER; note = 2 prime-O-methyl adenosine; note (original language) = 2'-O-甲基腺苷
  modified_base 15: mod_base = OTHER; note = 2 prime-O-methyl guanosine; note (original language) = 2'-O-甲基鸟苷
  modified_base 16: mod_base = OTHER; note = 2 prime-O-methyl adenosine; note (original language) = 2'-O-甲基腺苷
  modified_base 17: mod_base = OTHER; note = 2 prime-O-methyl guanosine; note (original language) = 2'-O-甲基鸟苷
  modified_base 18: mod_base = OTHER; note = 2 prime-O-methyl uridine; note (original language) = 2'-O-甲基尿苷
  modified_base 19: mod_base = OTHER; note = 2 prime-O-methyl adenosine; note (original language) = 2'-O-甲基腺苷
  modified_base 20: mod_base = OTHER; note = 2 prime-O-methyl cytidine; note (original language) = 2'-O-甲基胞苷
  modified_base 21: mod_base = OTHER; note = 2 prime-O-methyl adenosine conjugated to an N-[tris(GalNAc-alkyl)-amidodecanoyl)]-4-hydroxyprolinol (L96) ligand; note (original language) = 2'-O-甲基腺苷-缀合至N-[三(GalNAc-烷基)-酰胺癸酰基)]-4-羟基脯氨醇(L96)配体
  misc_feature 1^2: note = phosphorothioate linkage; note (original language) = 硫代磷酸酯连接
  misc_feature 2^3: note = phosphorothioate linkage; note (original language) = 硫代磷酸酯连接
gtcatccacaatgagagtaca

SEQ ID NO: 30 - RNA, 21 nt, synthetic construct
  source 1..21: mol_type = other RNA
  modified_base 1: mod_base = OTHER; note = 2 prime-O-methyl guanosine; note (original language) = 2'-O-甲基鸟苷
  modified_base 2: mod_base = OTHER; note = 2 prime-O-methyl uridine; note (original language) = 2'-O-甲基尿苷
  modified_base 3: mod_base = OTHER; note = 2 prime-O-methyl cytidine; note (original language) = 2'-O-甲基胞苷
  modified_base 4: mod_base = OTHER; note = 2 prime-O-methyl adenosine; note (original language) = 2'-O-甲基腺苷
  modified_base 5: mod_base = OTHER; note = 2 prime-O-methyl uridine; note (original language) = 2'-O-甲基尿苷
  modified_base 6: mod_base = OTHER; note = 2 prime-O-methyl cytidine; note (original language) = 2'-O-甲基胞苷
  modified_base 7: mod_base = OTHER; note = 2 prime fluorocytidine; note (original language) = 2'-氟代胞苷
  modified_base 8: mod_base = OTHER; note = 2 prime-O-methyl adenosine; note (original language) = 2'-O-甲基腺苷
  modified_base 9: mod_base = OTHER; note = 2 prime fluorocytidine; note (original language) = 2'-氟代胞苷
  modified_base 10..11: mod_base = OTHER; note = 2 prime fluoroadenosine; note (original language) = 2'-氟代腺苷
  modified_base 12: mod_base = OTHER; note = 2 prime-O-methyl uridine; note (original language) = 2'-O-甲基尿苷
  modified_base 13: mod_base = OTHER; note = 2 prime-O-methyl guanosine; note (original language) = 2'-O-甲基鸟苷
  modified_base 14: mod_base = OTHER; note = 2 prime-O-methyl adenosine; note (original language) = 2'-O-甲基腺苷
  modified_base 15: mod_base = OTHER; note = 2 prime-O-methyl guanosine; note (original language) = 2'-O-甲基鸟苷
  modified_base 16: mod_base = OTHER; note = 2 prime-O-methyl adenosine; note (original language) = 2'-O-甲基腺苷
  modified_base 17: mod_base = OTHER; note = 2 prime-O-methyl guanosine; note (original language) = 2'-O-甲基鸟苷
  modified_base 18: mod_base = OTHER; note = 2 prime-O-methyl uridine; note (original language) = 2'-O-甲基尿苷
  modified_base 19: mod_base = OTHER; note = 2 prime-O-methyl adenosine; note (original language) = 2'-O-甲基腺苷
  modified_base 20: mod_base = OTHER; note = 2 prime-O-methyl cytidine; note (original language) = 2'-O-甲基胞苷
  modified_base 21: mod_base = OTHER; note = 2 prime-O-methyl cytidine conjugated to an N-[tris(GalNAc-alkyl)-amidodecanoyl)]-4-hydroxyprolinol (L96) ligand; note (original language) = 2'-O-甲基胞苷-缀合至N-[三(GalNAc-烷基)-酰胺癸酰基)]-4-羟基脯氨醇(L96)配体
  misc_feature 1^2: note = phosphorothioate linkage; note (original language) = 硫代磷酸酯连接
  misc_feature 2^3: note = phosphorothioate linkage; note (original language) = 硫代磷酸酯连接
gtcatccacaatgagagtacc

SEQ ID NO: 31 - RNA, 21 nt, synthetic construct
  source 1..21: mol_type = other RNA
  modified_base 1: mod_base = OTHER; note = 2 prime-O-methyl guanosine; note (original language) = 2'-O-甲基鸟苷
  modified_base 2: mod_base = OTHER; note = 2 prime-O-methyl cytidine; note (original language) = 2'-O-甲基胞苷
  modified_base 3: mod_base = OTHER; note = 2 prime-O-methyl uridine; note (original language) = 2'-O-甲基尿苷
  modified_base 4: mod_base = OTHER; note = 2 prime-O-methyl guanosine; note (original language) = 2'-O-甲基鸟苷
  modified_base 5: mod_base = OTHER; note = 2 prime-O-methyl adenosine; note (original language) = 2'-O-甲基腺苷
  modified_base 6: mod_base = OTHER; note = 2 prime-O-methyl guanosine; note (original language) = 2'-O-甲基鸟苷
  modified_base 7: mod_base = OTHER; note = 2 prime fluoroadenosine; note (original language) = 2'-氟代腺苷
  modified_base 8: mod_base = OTHER; note = 2 prime-O-methyl adenosine; note (original language) = 2'-O-甲基腺苷
  modified_base 9: mod_base = OTHER; note = 2 prime fluoroguanosine; note (original language) = 2'-氟代鸟苷
  modified_base 10: mod_base = OTHER; note = 2 prime fluoroadenosine; note (original language) = 2'-氟代腺苷
  modified_base 11: mod_base = OTHER; note = 2 prime fluorouridine; note (original language) = 2'-氟代尿苷
  modified_base 12: mod_base = OTHER; note = 2 prime-O-methyl uridine; note (original language) = 2'-O-甲基尿苷
  modified_base 13: mod_base = OTHER; note = 2 prime-O-methyl guanosine; note (original language) = 2'-O-甲基鸟苷
  modified_base 14: mod_base = OTHER; note = 2 prime-O-methyl adenosine; note (original language) = 2'-O-甲基腺苷
  modified_base 15: mod_base = OTHER; note = 2 prime-O-methyl cytidine; note (original language) = 2'-O-甲基胞苷
  modified_base 16: mod_base = OTHER; note = 2 prime-O-methyl adenosine; note (original language) = 2'-O-甲基腺苷
  modified_base 17..18: mod_base = OTHER; note = 2 prime-O-methyl guanosine; note (original language) = 2'-O-甲基鸟苷
  modified_base 19..20: mod_base = OTHER; note = 2 prime-O-methyl uridine; note (original language) = 2'-O-甲基尿苷
  modified_base 21: mod_base = OTHER; note = 2 prime-O-methyl cytidine conjugated to an N-[tris(GalNAc-alkyl)-amidodecanoyl)]-4-hydroxyprolinol (L96) ligand; note (original language) = 2'-O-甲基胞苷-缀合至N-[三(GalNAc-烷基)-酰胺癸酰基)]-4-羟基脯氨醇(L96)配体
  misc_feature 1^2: note = phosphorothioate linkage; note (original language) = 硫代磷酸酯连接
  misc_feature 2^3: note = phosphorothioate linkage; note (original language) = 硫代磷酸酯连接
gctgagaagattgacaggttc

SEQ ID NO: 32 - RNA, 21 nt, synthetic construct
  source 1..21: mol_type = other RNA
  modified_base 1: mod_base = OTHER; note = 2 prime-O-methyl cytidine; note (original language) = 2'-O-甲基胞苷
  modified_base 2: mod_base = OTHER; note = 2 prime-O-methyl uridine; note (original language) = 2'-O-甲基尿苷
  modified_base 3: mod_base = OTHER; note = 2 prime-O-methyl guanosine; note (original language) = 2'-O-甲基鸟苷
  modified_base 4: mod_base = OTHER; note = 2 prime-O-methyl adenosine; note (original language) = 2'-O-甲基腺苷
  modified_base 5: mod_base = OTHER; note = 2 prime-O-methyl guanosine; note (original language) = 2'-O-甲基鸟苷
  modified_base 6: mod_base = OTHER; note = 2 prime-O-methyl adenosine; note (original language) = 2'-O-甲基腺苷
  modified_base 7: mod_base = OTHER; note = 2 prime fluoroadenosine; note (original language) = 2'-氟代腺苷
  modified_base 8: mod_base = OTHER; note = 2 prime-O-methyl guanosine; note (original language) = 2'-O-甲基鸟苷
  modified_base 9: mod_base = OTHER; note = 2 prime fluoroadenosine; note (original language) = 2'-氟代腺苷
  modified_base 10..11: mod_base = OTHER; note = 2 prime fluorouridine; note (original language) = 2'-氟代尿苷
  modified_base 12: mod_base = OTHER; note = 2 prime-O-methyl guanosine; note (original language) = 2'-O-甲基鸟苷
  modified_base 13: mod_base = OTHER; note = 2 prime-O-methyl adenosine; note (original language) = 2'-O-甲基腺苷
  modified_base 14: mod_base = OTHER; note = 2 prime-O-methyl cytidine; note (original language) = 2'-O-甲基胞苷
  modified_base 15: mod_base = OTHER; note = 2 prime-O-methyl adenosine; note (original language) = 2'-O-甲基腺苷
  modified_base 16..17: mod_base = OTHER; note = 2 prime-O-methyl guanosine; note (original language) = 2'-O-甲基鸟苷
  modified_base 18..19: mod_base = OTHER; note = 2 prime-O-methyl uridine; note (original language) = 2'-O-甲基尿苷
  modified_base 20: mod_base = OTHER; note = 2 prime-O-methyl cytidine; note (original language) = 2'-O-甲基胞苷
  modified_base 21: mod_base = OTHER; note = 2 prime-O-methyl adenosine conjugated to an N-[tris(GalNAc-alkyl)-amidodecanoyl)]-4-hydroxyprolinol (L96) ligand; note (original language) = 2'-O-甲基腺苷-缀合至N-[三(GalNAc-烷基)-酰胺癸酰基)]-4-羟基脯氨醇(L96)配体
  misc_feature 1^2: note = phosphorothioate linkage; note (original language) = 硫代磷酸酯连接
  misc_feature 2^3: note = phosphorothioate linkage; note (original language) = 硫代磷酸酯连接
ctgagaagattgacaggttca

SEQ ID NO: 33 - RNA, 21 nt, synthetic construct
  source 1..21: mol_type = other RNA
  modified_base 1..2: mod_base = OTHER; note = 2 prime-O-methyl cytidine; note (original language) = 2'-O-甲基胞苷
  modified_base 3: mod_base = OTHER; note = 2 prime-O-methyl uridine; note (original language) = 2'-O-甲基尿苷
  modified_base 4: mod_base = OTHER; note = 2 prime-O-methyl guanosine; note (original language) = 2'-O-甲基鸟苷
  modified_base 5..6: mod_base = OTHER; note = 2 prime-O-methyl uridine; note (original language) = 2'-O-甲基尿苷
  modified_base 7: mod_base = OTHER; note = 2 prime fluorouridine; note (original language) = 2'-氟代尿苷
  modified_base 8: mod_base = OTHER; note = 2 prime-O-methyl guanosine; note (original language) = 2'-O-甲基鸟苷
  modified_base 9: mod_base = OTHER; note = 2 prime fluorocytidine; note (original language) = 2'-氟代胞苷
  modified_base 10: mod_base = OTHER; note = 2 prime fluorouridine; note (original language) = 2'-氟代尿苷
  modified_base 11: mod_base = OTHER; note = 2 prime fluoroguanosine; note (original language) = 2'-氟代鸟苷
  modified_base 12: mod_base = OTHER; note = 2 prime-O-methyl uridine; note (original language) = 2'-O-甲基尿苷
  modified_base 13: mod_base = OTHER; note = 2 prime-O-methyl guanosine; note (original language) = 2'-O-甲基鸟苷
  modified_base 14: mod_base = OTHER; note = 2 prime-O-methyl uridine; note (original language) = 2'-O-甲基尿苷
  modified_base 15: mod_base = OTHER; note = 2 prime-O-methyl adenosine; note (original language) = 2'-O-甲基腺苷
  modified_base 16: mod_base = OTHER; note = 2 prime-O-methyl uridine; note (original language) = 2'-O-甲基尿苷
  modified_base 17: mod_base = OTHER; note = 2 prime-O-methyl guanosine; note (original language) = 2'-O-甲基鸟苷
  modified_base 18: mod_base = OTHER; note = 2 prime-O-methyl adenosine; note (original language) = 2'-O-甲基腺苷
  modified_base 19: mod_base = OTHER; note = 2 prime-O-methyl uridine; note (original language) = 2'-O-甲基尿苷
  modified_base 20: mod_base = OTHER; note = 2 prime-O-methyl cytidine; note (original language) = 2'-O-甲基胞苷
  modified_base 21: mod_base = OTHER; note = 2 prime-O-methyl adenosine conjugated to an N-[tris(GalNAc-alkyl)-amidodecanoyl)]-4-hydroxyprolinol (L96) ligand; note (original language) = 2'-O-甲基腺苷-缀合至N-[三(GalNAc-烷基)-酰胺癸酰基)]-4-羟基脯氨醇(L96)配体
  misc_feature 1^2: note = phosphorothioate linkage; note (original language) = 硫代磷酸酯连接
  misc_feature 2^3: note = phosphorothioate linkage; note (original language) = 硫代磷酸酯连接
cctgtttgctgtgtatgatca

SEQ ID NO: 34 - RNA, 21 nt, synthetic construct
  source 1..21: mol_type = other RNA
  modified_base 1..2: mod_base = OTHER; note = 2 prime-O-methyl guanosine; note (original language) = 2'-O-甲基鸟苷
  modified_base 3: mod_base = OTHER; note = 2 prime-O-methyl adenosine; note (original language) = 2'-O-甲基腺苷
  modified_base 4: mod_base = OTHER; note = 2 prime-O-methyl cytidine; note (original language) = 2'-O-甲基胞苷
  modified_base 5..6: mod_base = OTHER; note = 2 prime-O-methyl adenosine; note (original language) = 2'-O-甲基腺苷
  modified_base 7: mod_base = OTHER; note = 2 prime fluoroadenosine; note (original language) = 2'-氟代腺苷
  modified_base 8: mod_base = OTHER; note = 2 prime-O-methyl uridine; note (original language) = 2'-O-甲基尿苷
  modified_base 9: mod_base = OTHER; note = 2 prime fluorocytidine; note (original language) = 2'-氟代胞苷
  modified_base 10: mod_base = OTHER; note = 2 prime fluoroadenosine; note (original language) = 2'-氟代腺苷
  modified_base 11: mod_base = OTHER; note = 2 prime fluoroguanosine; note (original language) = 2'-氟代鸟苷
  modified_base 12: mod_base = OTHER; note = 2 prime-O-methyl cytidine; note (original language) = 2'-O-甲基胞苷
  modified_base 13: mod_base = OTHER; note = 2 prime-O-methyl guanosine; note (original language) = 2'-O-甲基鸟苷
  modified_base 14: mod_base = OTHER; note = 2 prime-O-methyl adenosine; note (original language) = 2'-O-甲基腺苷
  modified_base 13: mod_base = OTHER; note = 2 prime-O-methyl guanosine; note (original language) = 2'-O-甲基鸟苷
  modified_base 15: mod_base = OTHER; note = 2 prime-O-methyl uridine; note (original language) = 2'-O-甲基尿苷
  modified_base 16: mod_base = OTHER; note = 2 prime-O-methyl guanosine; note (original language) = 2'-O-甲基鸟苷
  modified_base 17: mod_base = OTHER; note = 2 prime-O-methyl uridine; note (original language) = 2'-O-甲基尿苷
  modified_base 18: mod_base = OTHER; note = 2 prime-O-methyl guanosine; note (original language) = 2'-O-甲基鸟苷
  modified_base 19: mod_base = OTHER; note = 2 prime-O-methyl uridine; note (original language) = 2'-O-甲基尿苷
  modified_base 20: mod_base = OTHER; note = 2 prime-O-methyl cytidine; note (original language) = 2'-O-甲基胞苷
  modified_base 21: mod_base = OTHER; note = 2 prime-O-methyl adenosine conjugated to an N-[tris(GalNAc-alkyl)-amidodecanoyl)]-4-hydroxyprolinol (L96) ligand; note (original language) = 2'-O-甲基腺苷-缀合至N-[三(GalNAc-烷基)-酰胺癸酰基)]-4-羟基脯氨醇(L96)配体
  misc_feature 1^2: note = phosphorothioate linkage; note (original language) = 硫代磷酸酯连接
  misc_feature 2^3: note = phosphorothioate linkage; note (original language) = 硫代磷酸酯连接
ggacaaatcagcgatgtgtca

SEQ ID NO: 35 - RNA, 21 nt, synthetic construct
  source 1..21: mol_type = other RNA
  modified_base 1: mod_base = OTHER; note = 2 prime-O-methyl cytidine; note (original language) = 2'-O-甲基胞苷
  modified_base 2: mod_base = OTHER; note = 2 prime-O-methyl adenosine; note (original language) = 2'-O-甲基腺苷
  modified_base 3: mod_base = OTHER; note = 2 prime-O-methyl guanosine; note (original language) = 2'-O-甲基鸟苷
  modified_base 4: mod_base = OTHER; note = 2 prime-O-methyl uridine; note (original language) = 2'-O-甲基尿苷
  modified_base 5: mod_base = OTHER; note = 2 prime-O-methyl cytidine; note (original language) = 2'-O-甲基胞苷
  modified_base 6: mod_base = OTHER; note = 2 prime-O-methyl uridine; note (original language) = 2'-O-甲基尿苷
  modified_base 7: mod_base = OTHER; note = 2 prime fluorocytidine; note (original language) = 2'-氟代胞苷
  modified_base 8: mod_base = OTHER; note = 2 prime-O-methyl cytidine; note (original language) = 2'-O-甲基胞苷
  modified_base 9: mod_base = OTHER; note = 2 prime fluorocytidine; note (original language) = 2'-氟代胞苷
  modified_base 10: mod_base = OTHER; note = 2 prime fluoroadenosine; note (original language) = 2'-氟代腺苷
  modified_base 11: mod_base = OTHER; note = 2 prime fluorocytidine; note (original language) = 2'-氟代胞苷
  modified_base 12: mod_base = OTHER; note = 2 prime-O-methyl cytidine; note (original language) = 2'-O-甲基胞苷
  modified_base 13..16: mod_base = OTHER; note = 2 prime-O-methyl uridine; note (original language) = 2'-O-甲基尿苷
  modified_base 17: mod_base = OTHER; note = 2 prime-O-methyl cytidine; note (original language) = 2'-O-甲基胞苷
  modified_base 18..19: mod_base = OTHER; note = 2 prime-O-methyl uridine; note (original language) = 2'-O-甲基尿苷
  modified_base 20: mod_base = OTHER; note = 2 prime-O-methyl cytidine; note (original language) = 2'-O-甲基胞苷
  modified_base 21: mod_base = OTHER; note = 2 prime-O-methyl uridine conjugated to an N-[tris(GalNAc-alkyl)-amidodecanoyl)]-4-hydroxyprolinol (L96) ligand; note (original language) = 2'-O-甲基尿苷-缀合至N-[三(GalNAc-烷基)-酰胺癸酰基)]-4-羟基脯氨醇(L96)配体
  misc_feature 1^2: note = phosphorothioate linkage; note (original language) = 硫代磷酸酯连接
  misc_feature 2^3: note = phosphorothioate linkage; note (original language) = 硫代磷酸酯连接
cagtctcccaccttttcttct

SEQ ID NO: 36 - RNA, 21 nt, synthetic construct
  source 1..21: mol_type = other RNA
  modified_base 1: mod_base = OTHER; note = 2 prime-O-methyl cytidine; note (original language) = 2'-O-甲基胞苷
  modified_base 2: mod_base = OTHER; note = 2 prime-O-methyl uridine; note (original language) = 2'-O-甲基尿苷
  modified_base 3..5: mod_base = OTHER; note = 2 prime-O-methyl cytidine; note (original language) = 2'-O-甲基胞苷
  modified_base 6: mod_base = OTHER; note = 2 prime-O-methyl adenosine; note (original language) = 2'-O-甲基腺苷
  modified_base 7: mod_base = OTHER; note = 2 prime fluorocytidine; note (original language) = 2'-氟代胞苷
  modified_base 8: mod_base = OTHER; note = 2 prime-O-methyl cytidine; note (original language) = 2'-O-甲基胞苷
  modified_base 9..11: mod_base = OTHER; note = 2 prime fluorouridine; note (original language) = 2'-氟代尿苷
  modified_base 12: mod_base = OTHER; note = 2 prime-O-methyl uridine; note (original language) = 2'-O-甲基尿苷
  modified_base 13: mod_base = OTHER; note = 2 prime-O-methyl cytidine; note (original language) = 2'-O-甲基胞苷
  modified_base 14..15: mod_base = OTHER; note = 2 prime-O-methyl uridine; note (original language) = 2'-O-甲基尿苷
  modified_base 16: mod_base = OTHER; note = 2 prime-O-methyl cytidine; note (original language) = 2'-O-甲基胞苷
  modified_base 17: mod_base = OTHER; note = 2 prime-O-methyl uridine; note (original language) = 2'-O-甲基尿苷
  modified_base 18..19: mod_base = OTHER; note = 2 prime-O-methyl adenosine; note (original language) = 2'-O-甲基腺苷
  modified_base 20: mod_base = OTHER; note = 2 prime-O-methyl uridine; note (original language) = 2'-O-甲基尿苷
  modified_base 21: mod_base = OTHER; note = 2 prime-O-methyl guanosine conjugated to an N-[tris(GalNAc-alkyl)-amidodecanoyl)]-4-hydroxyprolinol (L96) ligand; note (original language) = 2'-O-甲基鸟苷-缀合至N-[三(GalNAc-烷基)-酰胺癸酰基)]-4-羟基脯氨醇(L96)配体
  misc_feature 1^2: note = phosphorothioate linkage; note (original language) = 硫代磷酸酯连接
  misc_feature 2^3: note = phosphorothioate linkage; note (original language) = 硫代磷酸酯连接
ctcccaccttttcttctaatg

SEQ ID NO: 37 - RNA, 21 nt, synthetic construct
  source 1..21: mol_type = other RNA
  modified_base 1: mod_base = OTHER; note = 2 prime-O-methyl cytidine; note (original language) = 2'-O-甲基胞苷
  modified_base 2..3: mod_base = OTHER; note = 2 prime-O-methyl uridine; note (original language) = 2'-O-甲基尿苷
  modified_base 4: mod_base = OTHER; note = 2 prime-O-methyl cytidine; note (original language) = 2'-O-甲基胞苷
  modified_base 5: mod_base = OTHER; note = 2 prime-O-methyl uridine; note (original language) = 2'-O-甲基尿苷
  modified_base 6: mod_base = OTHER; note = 2 prime-O-methyl adenosine; note (original language) = 2'-O-甲基腺苷
  modified_base 7: mod_base = OTHER; note = 2 prime fluoroadenosine; note (original language) = 2'-氟代腺苷
  modified_base 8: mod_base = OTHER; note = 2 prime-O-methyl uridine; note (original language) = 2'-O-甲基尿苷
  modified_base 9: mod_base = OTHER; note = 2 prime fluoroguanosine; note (original language) = 2'-氟代鸟苷
  modified_base 10: mod_base = OTHER; note = 2 prime fluoroadenosine; note (original language) = 2'-氟代腺苷
  modified_base 11: mod_base = OTHER; note = 2 prime fluoroguanosine; note (original language) = 2'-氟代鸟苷
  modified_base 12: mod_base = OTHER; note = 2 prime-O-methyl uridine; note (original language) = 2'-O-甲基尿苷
  modified_base 13: mod_base = OTHER; note = 2 prime-O-methyl cytidine; note (original language) = 2'-O-甲基胞苷
  modified_base 14: mod_base = OTHER; note = 2 prime-O-methyl guanosine; note (original language) = 2'-O-甲基鸟苷
  modified_base 15: mod_base = OTHER; note = 2 prime-O-methyl adenosine; note (original language) = 2'-O-甲基腺苷
  modified_base 16: mod_base = OTHER; note = 2 prime-O-methyl cytidine; note (original language) = 2'-O-甲基胞苷
  modified_base 17..19: mod_base = OTHER; note = 2 prime-O-methyl uridine; note (original language) = 2'-O-甲基尿苷
  modified_base 20: mod_base = OTHER; note = 2 prime-O-methyl guanosine; note (original language) = 2'-O-甲基鸟苷
  modified_base 21: mod_base = OTHER; note = 2 prime-O-methyl adenosine conjugated to an N-[tris(GalNAc-alkyl)-amidodecanoyl)]-4-hydroxyprolinol (L96) ligand; note (original language) = '-O-甲基腺苷-缀合至N-[三(GalNAc-烷基)-酰胺癸酰基)]-4-羟基脯氨醇(L96)配体
  misc_feature 1^2: note = phosphorothioate linkage; note (original language) = 硫代磷酸酯连接
  misc_feature 2^3: note = phosphorothioate linkage; note (original language) = 硫代磷酸酯连接
cttctaatgagtcgactttga

SEQ ID NO: 38 - RNA, 21 nt, synthetic construct
  source 1..21: mol_type = other RNA
  modified_base 1: mod_base = OTHER; note = 2 prime-O-methyl guanosine; note (original language) = 2'-O-甲基鸟苷
  modified_base 2..4: mod_base = OTHER; note = 2 prime-O-methyl uridine; note (original language) = 2'-O-甲基尿苷
  modified_base 5: mod_base = OTHER; note = 2 prime-O-methyl cytidine; note (original language) = 2'-O-甲基胞苷
  modified_base 6: mod_base = OTHER; note = 2 prime-O-methyl uridine; note (original language) = 2'-O-甲基尿苷
  modified_base 7: mod_base = OTHER; note = 2 prime fluorocytidine; note (original language) = 2'-氟代胞苷
  modified_base 8: mod_base = OTHER; note = 2 prime-O-methyl cytidine; note (original language) = 2'-O-甲基胞苷
  modified_base 9..10: mod_base = OTHER; note = 2 prime fluorouridine; note (original language) = 2'-氟代尿苷
  modified_base 11: mod_base = OTHER; note = 2 prime fluoroguanosine; note (original language) = 2'-氟代鸟苷
  modified_base 12: mod_base = OTHER; note = 2 prime-O-methyl guanosine; note (original language) = 2'-O-甲基鸟苷
  modified_base 13: mod_base = OTHER; note = 2 prime-O-methyl uridine; note (original language) = 2'-O-甲基尿苷
  modified_base 14: mod_base = OTHER; note = 2 prime-O-methyl cytidine; note (original language) = 2'-O-甲基胞苷
  modified_base 15: mod_base = OTHER; note = 2 prime-O-methyl uridine; note (original language) = 2'-O-甲基尿苷
  modified_base 16..17: mod_base = OTHER; note = 2 prime-O-methyl adenosine; note (original language) = 2'-O-甲基腺苷
  modified_base 18: mod_base = OTHER; note = 2 prime-O-methyl guanosine; note (original language) = 2'-O-甲基鸟苷
  modified_base 19: mod_base = OTHER; note = 2 prime-O-methyl uridine; note (original language) = 2'-O-甲基尿苷
  modified_base 20: mod_base = OTHER; note = 2 prime-O-methyl guanosine; note (original language) = 2'-O-甲基鸟苷
  modified_base 21: mod_base = OTHER; note = 2 prime-O-methyl uridine conjugated to an N-[tris(GalNAc-alkyl)-amidodecanoyl)]-4-hydroxyprolinol (L96) ligand; note (original language) = 2'-O-甲基尿苷-缀合至N-[三(GalNAc-烷基)-酰胺癸酰基)]-4-羟基脯氨醇(L96)配体
  misc_feature 1^2: note = phosphorothioate linkage; note (original language) = 硫代磷酸酯连接
  misc_feature 2^3: note = phosphorothioate linkage; note (original language) = 硫代磷酸酯连接
gtttctccttggtctaagtgt

SEQ ID NO: 39 - RNA, 21 nt, synthetic construct
  source 1..21: mol_type = other RNA
  modified_base 1: mod_base = OTHER; note = 2 prime-O-methyl guanosine; note (original language) = 2'-O-甲基鸟苷
  modified_base 2: mod_base = OTHER; note = 2 prime-O-methyl cytidine; note (original language) = 2'-O-甲基胞苷
  modified_base 3..4: mod_base = OTHER; note = 2 prime-O-methyl uridine; note (original language) = 2'-O-甲基尿苷
  modified_base 5: mod_base = OTHER; note = 2 prime-O-methyl guanosine; note (original language) = 2'-O-甲基鸟苷
  modified_base 6: mod_base = OTHER; note = 2 prime-O-methyl uridine; note (original language) = 2'-O-甲基尿苷
  modified_base 7: mod_base = OTHER; note = 2 prime fluorouridine; note (original language) = 2'-氟代尿苷
  modified_base 8: mod_base = OTHER; note = 2 prime-O-methyl uridine; note (original language) = 2'-O-甲基尿苷
  modified_base 9: mod_base = OTHER; note = 2 prime fluoroguanosine; note (original language) = 2'-氟代鸟苷
  modified_base 10: mod_base = OTHER; note = 2 prime fluorouridine; note (original language) = 2'-氟代尿苷
  modified_base 11: mod_base = OTHER; note = 2 prime fluoroguanosine; note (original language) = 2'-氟代鸟苷
  modified_base 12..14: mod_base = OTHER; note = 2 prime-O-methyl adenosine; note (original language) = 2'-O-甲基腺苷
  modified_base 15: mod_base = OTHER; note = 2 prime-O-methyl cytidine; note (original language) = 2'-O-甲基胞苷
  modified_base 16..20: mod_base = OTHER; note = 2 prime-O-methyl adenosine; note (original language) = 2'-O-甲基腺苷
  modified_base 21: mod_base = OTHER; note = 2 prime-O-methyl adenosine conjugated to an N-[tris(GalNAc-alkyl)-amidodecanoyl)]-4-hydroxyprolinol (L96) ligand; note (original language) = 2'-O-甲基腺苷-缀合至N-[三(GalNAc-烷基)-酰胺癸酰基)]-4-羟基脯氨醇(L96)配体
  misc_feature 1^2: note = phosphorothioate linkage; note (original language) = 硫代磷酸酯连接
  misc_feature 2^3: note = phosphorothioate linkage; note (original language) = 硫代磷酸酯连接
gcttgtttgtgaaacaaaaaa

SEQ ID NO: 40 - RNA, 21 nt, synthetic construct
  source 1..21: mol_type = other RNA
gtgccttgatcttggacttcc

SEQ ID NO: 41 - RNA, 23 nt, synthetic construct
  source 1..23: mol_type = other RNA
ggaagtccaagatcaaggcactg

SEQ ID NO: 42 - RNA, 21 nt, synthetic construct
  source 1..21: mol_type = other RNA
ccttgatcttggacttccagc

SEQ ID NO: 43 - RNA, 23 nt, synthetic construct
  source 1..23: mol_type = other RNA
gctggaagtccaagatcaaggca

SEQ ID NO: 44 - RNA, 21 nt, synthetic construct
  source 1..21: mol_type = other RNA
cttcatacctgctccaattca

SEQ ID NO: 45 - RNA, 23 nt, synthetic construct
  source 1..23: mol_type = other RNA
tgaattggagcaggtatgaaggt

SEQ ID NO: 46 - RNA, 21 nt, synthetic construct
  source 1..21: mol_type = other RNA
catcccctgtggatgaaaagg

SEQ ID NO: 47 - RNA, 23 nt, synthetic construct
  source 1..23: mol_type = other RNA
ccttttcatccacaggggatgtc

SEQ ID NO: 48 - RNA, 21 nt, synthetic construct
  source 1..21: mol_type = other RNA
gctagtcgctgcaaaacttga

SEQ ID NO: 49 - RNA, 23 nt, synthetic construct
  source 1..23: mol_type = other RNA
tcaagttttgcagcgactagcac

SEQ ID NO: 50 - RNA, 21 nt, synthetic construct
  source 1..21: mol_type = other RNA
gtcgctgcaaaacttgacacc

SEQ ID NO: 51 - RNA, 23 nt, synthetic construct
  source 1..23: mol_type = other RNA
ggtgtcaagttttgcagcgacta

SEQ ID NO: 52 - RNA, 21 nt, synthetic construct
  source 1..21: mol_type = other RNA
ctgcaaaacttgacaccgaag

SEQ ID NO: 53 - RNA, 23 nt, synthetic construct
  source 1..23: mol_type = other RNA
cttcggtgtcaagttttgcagcg

SEQ ID NO: 54 - RNA, 21 nt, synthetic construct
  source 1..21: mol_type = other RNA
caaaacttgacaccgaagaca

SEQ ID NO: 55 - RNA, 23 nt, synthetic construct
  source 1..23: mol_type = other RNA
tgtcttcggtgtcaagttttgca

SEQ ID NO: 56 - RNA, 21 nt, synthetic construct
  source 1..21: mol_type = other RNA
ggcttccgtatatatggcatg

SEQ ID NO: 57 - RNA, 23 nt, synthetic construct
  source 1..23: mol_type = other RNA
catgccatatatacggaagccca

SEQ ID NO: 58 - RNA, 21 nt, synthetic construct
  source 1..21: mol_type = other RNA
gcttccgtatatatggcatgc

SEQ ID NO: 59 - RNA, 23 nt, synthetic construct
  source 1..23: mol_type = other RNA
gcatgccatatatacggaagccc

SEQ ID NO: 60 - RNA, 21 nt, synthetic construct
  source 1..21: mol_type = other RNA
gttccttggaaggacaagaac

SEQ ID NO: 61 - RNA, 23 nt, synthetic construct
  source 1..23: mol_type = other RNA
gttcttgtccttccaaggaacac

SEQ ID NO: 62 - RNA, 21 nt, synthetic construct
  source 1..21: mol_type = other RNA
ctctggacttcacagaactgg

SEQ ID NO: 63 - RNA, 23 nt, synthetic construct
  source 1..23: mol_type = other RNA
ccagttctgtgaagtccagagag

SEQ ID NO: 64 - RNA, 21 nt, synthetic construct
  source 1..21: mol_type = other RNA
ggacttcacagaactggatgt

SEQ ID NO: 65 - RNA, 23 nt, synthetic construct
  source 1..23: mol_type = other RNA
acatccagttctgtgaagtccag

SEQ ID NO: 66 - RNA, 21 nt, synthetic construct
  source 1..21: mol_type = other RNA
cttcacagaactggatgttgc

SEQ ID NO: 67 - RNA, 23 nt, synthetic construct
  source 1..23: mol_type = other RNA
gcaacatccagttctgtgaagtc

SEQ ID NO: 68 - RNA, 21 nt, synthetic construct
  source 1..21: mol_type = other RNA
gctgctgagaagattgacagg

SEQ ID NO: 69 - RNA, 23 nt, synthetic construct
  source 1..23: mol_type = other RNA
cctgtcaatcttctcagcagcaa

SEQ ID NO: 70 - RNA, 21 nt, synthetic construct
  source 1..21: mol_type = other RNA
gctgagaagattgacaggttc

SEQ ID NO: 71 - RNA, 23 nt, synthetic construct
  source 1..23: mol_type = other RNA
gaacctgtcaatcttctcagcag

SEQ ID NO: 72 - RNA, 21 nt, synthetic construct
  source 1..21: mol_type = other RNA
ctgagaagattgacaggttca

SEQ ID NO: 73 - RNA, 23 nt, synthetic construct
  source 1..23: mol_type = other RNA
tgaacctgtcaatcttctcagca

SEQ ID NO: 74 - RNA, 21 nt, synthetic construct
  source 1..21: mol_type = other RNA
gacaacagcacctcagtgtct

SEQ ID NO: 75 - RNA, 23 nt, synthetic construct
  source 1..23: mol_type = other RNA
agacactgaggtgctgttgtcca

SEQ ID NO: 76 - RNA, 21 nt, synthetic construct
  source 1..21: mol_type = other RNA
gtgacatccaggacaacttct

SEQ ID NO: 77 - RNA, 23 nt, synthetic construct
  source 1..23: mol_type = other RNA
agaagttgtcctggatgtcactc

SEQ ID NO: 78 - RNA, 21 nt, synthetic construct
  source 1..21: mol_type = other RNA
ggtctcactttccagcaaaac

SEQ ID NO: 79 - RNA, 23 nt, synthetic construct
  source 1..23: mol_type = other RNA
gttttgctggaaagtgagaccct

SEQ ID NO: 80 - RNA, 21 nt, synthetic construct
  source 1..21: mol_type = other RNA
gtctcactttccagcaaaact

SEQ ID NO: 81 - RNA, 23 nt, synthetic construct
  source 1..23: mol_type = other RNA
agttttgctggaaagtgagaccc

SEQ ID NO: 82 - RNA, 21 nt, synthetic construct
  source 1..21: mol_type = other RNA
ctttccagcaaaactccctca

SEQ ID NO: 83 - RNA, 23 nt, synthetic construct
  source 1..23: mol_type = other RNA
tgagggagttttgctggaaagtg

SEQ ID NO: 84 - RNA, 21 nt, synthetic construct
  source 1..21: mol_type = other RNA
cagcaaaactccctcaactgg

SEQ ID NO: 85 - RNA, 23 nt, synthetic construct
  source 1..23: mol_type = other RNA
ccagttgagggagttttgctgga

SEQ ID NO: 86 - RNA, 21 nt, synthetic construct
  source 1..21: mol_type = other RNA
ggtgctgcaaggatcttatga

SEQ ID NO: 87 - RNA, 23 nt, synthetic construct
  source 1..23: mol_type = other RNA
tcataagatccttgcagcaccag

SEQ ID NO: 88 - RNA, 21 nt, synthetic construct
  source 1..21: mol_type = other RNA
gatcttatgacctgcaggacc

SEQ ID NO: 89 - RNA, 23 nt, synthetic construct
  source 1..23: mol_type = other RNA
ggtcctgcaggtcataagatcct

SEQ ID NO: 90 - RNA, 21 nt, synthetic construct
  source 1..21: mol_type = other RNA
cctgcaaaaattgagcaatga

SEQ ID NO: 91 - RNA, 23 nt, synthetic construct
  source 1..23: mol_type = other RNA
tcattgctcaatttttgcaggtt

SEQ ID NO: 92 - RNA, 21 nt, synthetic construct
  source 1..21: mol_type = other RNA
gaggtgctgaacagcattttt

SEQ ID NO: 93 - RNA, 23 nt, synthetic construct
  source 1..23: mol_type = other RNA
aaaaatgctgttcagcacctccc

SEQ ID NO: 94 - RNA, 21 nt, synthetic construct
  source 1..21: mol_type = other RNA
ctacccaacagcttaacaagc

SEQ ID NO: 95 - RNA, 23 nt, synthetic construct
  source 1..23: mol_type = other RNA
gcttgttaagctgttgggtagac

SEQ ID NO: 96 - RNA, 21 nt, synthetic construct
  source 1..21: mol_type = other RNA
ccaacagcttaacaagcctga

SEQ ID NO: 97 - RNA, 23 nt, synthetic construct
  source 1..23: mol_type = other RNA
tcaggcttgttaagctgttgggt

SEQ ID NO: 98 - RNA, 21 nt, synthetic construct
  source 1..21: mol_type = other RNA
ccattcctgtttgctgtgtat

SEQ ID NO: 99 - RNA, 23 nt, synthetic construct
  source 1..23: mol_type = other RNA
atacacagcaaacaggaatgggc

SEQ ID NO: 100 - RNA, 21 nt, synthetic construct
  source 1..21: mol_type = other RNA
cattcctgtttgctgtgtatg

SEQ ID NO: 101 - RNA, 23 nt, synthetic construct
  source 1..23: mol_type = other RNA
catacacagcaaacaggaatggg

SEQ ID NO: 102 - RNA, 21 nt, synthetic construct
  source 1..21: mol_type = other RNA
cctgtttgctgtgtatgatca

SEQ ID NO: 103 - RNA, 23 nt, synthetic construct
  source 1..23: mol_type = other RNA
tgatcatacacagcaaacaggaa

SEQ ID NO: 104 - RNA, 21 nt, synthetic construct
  source 1..21: mol_type = other RNA
gtatgatcaaagcgccactgc

SEQ ID NO: 105 - RNA, 23 nt, synthetic construct
  source 1..23: mol_type = other RNA
gcagtggcgctttgatcatacac

SEQ ID NO: 106 - RNA, 21 nt, synthetic construct
  source 1..21: mol_type = other RNA
ggacaaatcagcgatgtgtca

SEQ ID NO: 107 - RNA, 23 nt, synthetic construct
  source 1..23: mol_type = other RNA
tgacacatcgctgatttgtccgg

SEQ ID NO: 108 - RNA, 21 nt, synthetic construct
  source 1..21: mol_type = other RNA
cagtctcccaccttttcttct

SEQ ID NO: 109 - RNA, 23 nt, synthetic construct
  source 1..23: mol_type = other RNA
agaagaaaaggtgggagactggg

SEQ ID NO: 110 - RNA, 21 nt, synthetic construct
  source 1..21: mol_type = other RNA
ctcccaccttttcttctaatg

SEQ ID NO: 111 - RNA, 23 nt, synthetic construct
  source 1..23: mol_type = other RNA
cattagaagaaaaggtgggagac

SEQ ID NO: 112 - RNA, 21 nt, synthetic construct
  source 1..21: mol_type = other RNA
gtttctccttggtctaagtgt

SEQ ID NO: 113 - RNA, 23 nt, synthetic construct
  source 1..23: mol_type = other RNA
acacttagaccaaggagaaacgg

SEQ ID NO: 114 - RNA, 21 nt, synthetic construct
  source 1..21: mol_type = other RNA
catggagtgagcagtagaagc

SEQ ID NO: 115 - RNA, 23 nt, synthetic construct
  source 1..23: mol_type = other RNA
gcttctactgctcactccatgca

SEQ ID NO: 116 - RNA, 21 nt, synthetic construct
  source 1..21: mol_type = other RNA
ccagtttgctgggtttatttt

SEQ ID NO: 117 - RNA, 23 nt, synthetic construct
  source 1..23: mol_type = other RNA
aaaataaacccagcaaactggga

SEQ ID NO: 118 - RNA, 21 nt, synthetic construct
  source 1..21: mol_type = other RNA
gctgggtttattttagagaat

SEQ ID NO: 119 - RNA, 23 nt, synthetic construct
  source 1..23: mol_type = other RNA
attctctaaaataaacccagcaa

SEQ ID NO: 120 - RNA, 21 nt, synthetic construct
  source 1..21: mol_type = other RNA
ctgggtttattttagagaatg

SEQ ID NO: 121 - RNA, 23 nt, synthetic construct
  source 1..23: mol_type = other RNA
cattctctaaaataaacccagca

SEQ ID NO: 122 - RNA, 21 nt, synthetic construct
  source 1..21: mol_type = other RNA
gaggcaagaaccagtgtttag

SEQ ID NO: 123 - RNA, 23 nt, synthetic construct
  source 1..23: mol_type = other RNA
ctaaacactggttcttgcctccc

SEQ ID NO: 124 - RNA, 21 nt, synthetic construct
  source 1..21: mol_type = other RNA
cgggactactgttccaaaaag

SEQ ID NO: 125 - RNA, 23 nt, synthetic construct
  source 1..23: mol_type = other RNA
ctttttggaacagtagtcccgcg

SEQ ID NO: 126 - RNA, 21 nt, synthetic construct
  source 1..21: mol_type = other RNA
gactactgttccaaaaagaat

SEQ ID NO: 127 - RNA, 23 nt, synthetic construct
  source 1..23: mol_type = other RNA
attctttttggaacagtagtccc

SEQ ID NO: 128 - RNA, 21 nt, synthetic construct
  source 1..21: mol_type = other RNA
gttccaaaaagaattccaacc

SEQ ID NO: 129 - RNA, 23 nt, synthetic construct
  source 1..23: mol_type = other RNA
ggttggaattctttttggaacag

SEQ ID NO: 130 - RNA, 21 nt, synthetic construct
  source 1..21: mol_type = other RNA
caaaaagaattccaaccgacc

SEQ ID NO: 131 - RNA, 23 nt, synthetic construct
  source 1..23: mol_type = other RNA
ggtcggttggaattctttttgga

SEQ ID NO: 132 - RNA, 21 nt, synthetic construct
  source 1..21: mol_type = other RNA
cgaccagcttgtttgtgaaac

SEQ ID NO: 133 - RNA, 23 nt, synthetic construct
  source 1..23: mol_type = other RNA
gtttcacaaacaagctggtcggt

SEQ ID NO: 134 - RNA, 21 nt, synthetic construct
  source 1..21: mol_type = other RNA
ccagcttgtttgtgaaacaaa

SEQ ID NO: 135 - RNA, 23 nt, synthetic construct
  source 1..23: mol_type = other RNA
tttgtttcacaaacaagctggtc

SEQ ID NO: 136 - RNA, 21 nt, synthetic construct
  source 1..21: mol_type = other RNA
cagcttgtttgtgaaacaaaa

SEQ ID NO: 137 - RNA, 23 nt, synthetic construct
  source 1..23: mol_type = other RNA
ttttgtttcacaaacaagctggt

SEQ ID NO: 138 - RNA, 21 nt, synthetic construct
  source 1..21: mol_type = other RNA
gcttgtttgtgaaacaaaaaa

SEQ ID NO: 139 - RNA, 23 nt, synthetic construct
  source 1..23: mol_type = other RNA
ttttttgtttcacaaacaagctg

SEQ ID NO: 140 - RNA, 21 nt, synthetic construct
  source 1..21: mol_type = other RNA
cttttcaagttgagaacaaaa

SEQ ID NO: 141 - RNA, 23 nt, synthetic construct
  source 1..23: mol_type = other RNA
ttttgttctcaacttgaaaaggg

SEQ ID NO: 142 - RNA, 21 nt, synthetic construct
  source 1..21: mol_type = other RNA
gagaacaaaaattgggtttta

SEQ ID NO: 143 - RNA, 23 nt, synthetic construct
  source 1..23: mol_type = other RNA
taaaacccaatttttgttctcaa

SEQ ID NO: 144 - RNA, 21 nt, synthetic construct
  source 1..21: mol_type = other RNA
gcattgccttcggtttgtatt

SEQ ID NO: 145 - RNA, 23 nt, synthetic construct
  source 1..23: mol_type = other RNA
aatacaaaccgaaggcaatgcaa

SEQ ID NO: 146 - RNA, 21 nt, synthetic construct
  source 1..21: mol_type = other RNA
ccttcggtttgtatttagtgt

SEQ ID NO: 147 - RNA, 23 nt, synthetic construct
  source 1..23: mol_type = other RNA
acactaaatacaaaccgaaggca

SEQ ID NO: 148 - RNA, 21 nt, synthetic construct
  source 1..21: mol_type = other RNA
cggtttgtatttagtgtcttg

SEQ ID NO: 149 - RNA, 23 nt, synthetic construct
  source 1..23: mol_type = other RNA
caagacactaaatacaaaccgaa

SEQ ID NO: 150 - RNA, 21 nt, synthetic construct
  source 1..21: mol_type = other RNA
ggtttgtatttagtgtcttga

SEQ ID NO: 151 - RNA, 23 nt, synthetic construct
  source 1..23: mol_type = other RNA
tcaagacactaaatacaaaccga

SEQ ID NO: 152 - RNA, 21 nt, synthetic construct
  source 1..21: mol_type = other RNA
cttgaatgtaagaacatgacc

SEQ ID NO: 153 - RNA, 23 nt, synthetic construct
  source 1..23: mol_type = other RNA
ggtcatgttcttacattcaagac

SEQ ID NO: 154 - RNA, 21 nt, synthetic construct
  source 1..21: mol_type = other RNA
gaatgtaagaacatgacctcc

SEQ ID NO: 155 - RNA, 23 nt, synthetic construct
  source 1..23: mol_type = other RNA
ggaggtcatgttcttacattcaa

SEQ ID NO: 156 - RNA, 21 nt, synthetic construct
  source 1..21: mol_type = other RNA
gtaagaacatgacctccgtgt

SEQ ID NO: 157 - RNA, 23 nt, synthetic construct
  source 1..23: mol_type = other RNA
acacggaggtcatgttcttacat

SEQ ID NO: 158 - RNA, 21 nt, synthetic construct
  source 1..21: mol_type = other RNA
gtgtctgtaataccttagttt

SEQ ID NO: 159 - RNA, 23 nt, synthetic construct
  source 1..23: mol_type = other RNA
aaactaaggtattacagacacta

SEQ ID NO: 160 - RNA, 21 nt, synthetic construct
  source 1..21: mol_type = other RNA
gtctgtaataccttagttttt

SEQ ID NO: 161 - RNA, 23 nt, synthetic construct
  source 1..23: mol_type = other RNA
aaaaactaaggtattacagacac

SEQ ID NO: 162 - RNA, 21 nt, synthetic construct
  source 1..21: mol_type = other RNA
gcttgtgatttttgaacaata

SEQ ID NO: 163 - RNA, 23 nt, synthetic construct
  source 1..23: mol_type = other RNA
tattgttcaaaaatcacaagcat

SEQ ID NO: 164 - RNA, 21 nt, synthetic construct
  source 1..21: mol_type = other RNA
caatacgtgaaagatgcaagc

SEQ ID NO: 165 - RNA, 23 nt, synthetic construct
  source 1..23: mol_type = other RNA
gcttgcatctttcacgtattgtt

SEQ ID NO: 166 - RNA, 21 nt, synthetic construct
  source 1..21: mol_type = other RNA
gaaagatgcaagcacctgaat

SEQ ID NO: 167 - RNA, 23 nt, synthetic construct
  source 1..23: mol_type = other RNA
attcaggtgcttgcatctttcac

SEQ ID NO: 168 - RNA, 21 nt, synthetic construct
  source 1..21: mol_type = other RNA
gatgcaagcacctgaatttct

SEQ ID NO: 169 - RNA, 23 nt, synthetic construct
  source 1..23: mol_type = other RNA
agaaattcaggtgcttgcatctt

SEQ ID NO: 170 - RNA, 21 nt, synthetic construct
  source 1..21: mol_type = other RNA
cacctgaatttctgtttgaat

SEQ ID NO: 171 - RNA, 23 nt, synthetic construct
  source 1..23: mol_type = other RNA
attcaaacagaaattcaggtgct

SEQ ID NO: 172 - RNA, 21 nt, synthetic construct
  source 1..21: mol_type = other RNA
ctgtttgaatgcggaaccata

SEQ ID NO: 173 - RNA, 23 nt, synthetic construct
  source 1..23: mol_type = other RNA
tatggttccgcattcaaacagaa

SEQ ID NO: 174 - RNA, 21 nt, synthetic construct
  source 1..21: mol_type = other RNA
cggaaccatagctggttattt

SEQ ID NO: 175 - RNA, 23 nt, synthetic construct
  source 1..23: mol_type = other RNA
aaataaccagctatggttccgca

SEQ ID NO: 176 - RNA, 21 nt, synthetic construct
  source 1..21: mol_type = other RNA
ctggttatttctcccttgtgt

SEQ ID NO: 177 - RNA, 23 nt, synthetic construct
  source 1..23: mol_type = other RNA
acacaagggagaaataaccagct

SEQ ID NO: 178 - RNA, 21 nt, synthetic construct
  source 1..21: mol_type = other RNA
ggttatttctcccttgtgtta

SEQ ID NO: 179 - RNA, 23 nt, synthetic construct
  source 1..23: mol_type = other RNA
taacacaagggagaaataaccag

SEQ ID NO: 180 - RNA, 21 nt, synthetic construct
  source 1..21: mol_type = other RNA
cccttgtgttagtaataaacg

SEQ ID NO: 181 - RNA, 23 nt, synthetic construct
  source 1..23: mol_type = other RNA
cgtttattactaacacaagggag

SEQ ID NO: 182 - RNA, 21 nt, synthetic construct
  source 1..21: mol_type = other RNA
gtgttagtaataaacgtcttg

SEQ ID NO: 183 - RNA, 23 nt, synthetic construct
  source 1..23: mol_type = other RNA
caagacgtttattactaacacaa

SEQ ID NO: 184 - RNA, 21 nt, synthetic construct
  source 1..21: mol_type = other RNA
gccacaataagcctccaaaaa

SEQ ID NO: 185 - RNA, 23 nt, synthetic construct
  source 1..23: mol_type = other RNA
tttttggaggcttattgtggcaa

SEQ ID NO: 186 - RNA, 21 nt, synthetic construct
  source 1..21: mol_type = other RNA; note; note (original language) = NC对照组有义链
ttctccgaacgtgtcacgttt

SEQ ID NO: 187 - RNA, 21 nt, synthetic construct
  source 1..21: mol_type = other RNA; note; note (original language) = NC对照组反义链
acgtgacacgttcggagaatt

SEQ ID NO: 188 - RNA, 21 nt, synthetic construct
  source 1..21: mol_type = other RNA; note; note (original language) = 阳性对照AD85481有义链
gtcatccacaatgagagtaca

SEQ ID NO: 189 - RNA, 23 nt, synthetic construct
  source 1..23: mol_type = other RNA; note; note (original language) = 阳性对照AD85481反义链
tgtactctcattgtggatgacga

SEQ ID NO: 190 - DNA, 19 bp, synthetic construct
  source 1..19: mol_type = other DNA; note; note (original language) = 引物H-GAPDH-F
ggtcggagtcaacggattt

SEQ ID NO: 191 - DNA, 19 bp, synthetic construct
  source 1..19: mol_type = other DNA; note; note (original language) = 引物H-GAPDH-R
ccagcatcgccccacttga

SEQ ID NO: 192 - DNA, 20 bp, synthetic construct
  source 1..20: mol_type = other DNA; note; note (original language) = 引物H-AGT-F
tccagcctcactatgcctct

SEQ ID NO: 193 - DNA, 20 bp, synthetic construct
  source 1..20: mol_type = other DNA; note; note (original language) = 引物H-AGT-R
ggctctctctcatccgcttc

SEQ ID NO: 194 - RNA, 23 nt, synthetic construct
  source 1..23: mol_type = other RNA
  modified_base 6: mod_base = OTHER; note = thymidine-glycol nucleic acid (GNA) S-isomer((s)-GNA-T); note (original language) = 腺苷-乙二醇核酸 (GNA) S-异构体((s)-GNA-T)
  modified_base 1: mod_base = OTHER; note = 2 prime-O-methyl uridine; note (original language) = 2'-O-甲基尿苷
  modified_base 2: mod_base = OTHER; note = 2 prime fluoroguanosine; note (original language) = 2'-氟代鸟苷
  modified_base 3: mod_base = OTHER; note = 2 prime-O-methyl uridine; note (original language) = 2'-O-甲基尿苷
  modified_base 4: mod_base = OTHER; note = 2 prime-O-methyl adenosine; note (original language) = 2'-O-甲基腺苷
  modified_base 5: mod_base = OTHER; note = 2 prime-O-methyl cytidine; note (original language) = 2'-O-甲基胞苷
  modified_base 7: mod_base = OTHER; note = 2 prime-O-methyl cytidine; note (original language) = 2'-O-甲基胞苷
  modified_base 8: mod_base = OTHER; note = 2 prime-O-methyl uridine; note (original language) = 2'-O-甲基尿苷
  modified_base 9: mod_base = OTHER; note = 2 prime-O-methyl cytidine; note (original language) = 2'-O-甲基胞苷
  modified_base 10: mod_base = OTHER; note = 2 prime-O-methyl adenosine; note (original language) = 2'-O-甲基腺苷
  modified_base 11..12: mod_base = OTHER; note = 2 prime-O-methyl uridine; note (original language) = 2'-O-甲基尿苷
  modified_base 13: mod_base = OTHER; note = 2 prime-O-methyl guanosine; note (original language) = 2'-O-甲基鸟苷
  modified_base 14: mod_base = OTHER; note = 2 prime fluorouridine; note (original language) = 2'-氟代尿苷
  modified_base 15: mod_base = OTHER; note = 2 prime-O-methyl guanosine; note (original language) = 2'-O-甲基鸟苷
  modified_base 16: mod_base = OTHER; note = 2 prime fluoroguanosine; note (original language) = 2'-氟代鸟苷
  modified_base 17: mod_base = OTHER; note = 2 prime-O-methyl adenosine; note (original language) = 2'-O-甲基腺苷
  modified_base 18: mod_base = OTHER; note = 2 prime-O-methyl uridine; note (original language) = 2'-O-甲基尿苷
  modified_base 19: mod_base = OTHER; note = 2 prime-O-methyl guanosine; note (original language) = 2'-O-甲基鸟苷
  modified_base 20: mod_base = OTHER; note = 2 prime-O-methyl adenosine; note (original language) = 2'-O-甲基腺苷
  modified_base 21: mod_base = OTHER; note = 2 prime-O-methyl cytidine; note (original language) = 2'-O-甲基胞苷
  modified_base 22: mod_base = OTHER; note = 2 prime-O-methyl guanosine; note (original language) = 2'-O-甲基鸟苷
  modified_base 23: mod_base = OTHER; note = 2 prime-O-methyl adenosine; note (original language) = 2'-O-甲基腺苷
  misc_feature 1^2: note = phosphorothioate linkage; note (original language) = 硫代磷酸酯连接
  misc_feature 2^3: note = phosphorothioate linkage; note (original language) = 硫代磷酸酯连接
  misc_feature 21^22: note = phosphorothioate linkage; note (original language) = 硫代磷酸酯连接
  misc_feature 22^23: note = phosphorothioate linkage; note (original language) = 硫代磷酸酯连接
tgtactctcattgtggatgacga